European Patent Specification EP 3 535 290 B1, published January 10, 2024. Title: An engineered two-part cellular device for discovery and characterisation of T-cell receptor interaction with cognate antigen. Applicant: Genovie AB. The sequence listing filed with the application follows.

SEQUENCE LISTING (104 sequences)

SEQ ID NO: 1 - protein, 9 aa, Cytomegalovirus
  Analyte Antigenic Peptide
NLVPMVATV

SEQ ID NO: 2 - protein, 9 aa, Artificial Sequence
  Analyte Antigenic Peptide
VYALPLKML

SEQ ID NO: 3 - protein, 4 aa, Homo sapiens
  HCMV Antigen
NLVP

SEQ ID NO: 4 - protein, 4 aa, Homo sapiens
  HCMV Antigen
NLVP

SEQ ID NO: 5 - DNA, 6071 bp, Artificial Sequence
  pcDNA3.1_GFP vector V1.A.4
gacggatcgggagatctcccgatcccctatggtgcactctcagtacaatctgctctgatgccgcatagttaagccagtatctgctccctgcttgtgtgttggaggtcgctgagtagtgcgcgagcaaaatttaagctacaacaaggcaaggcttgaccgacaattgcatgaagaatctgcttagggttaggcgttttgcgctgcttcgcgatgtacgggccagatatacgcgttgacattgattattgactagttattaatagtaatcaattacggggtcattagttcatagcccatatatggagttccgcgttacataacttacggtaaatggcccgcctggctgaccgcccaacgacccccgcccattgacgtcaataatgacgtatgttcccatagtaacgccaatagggactttccattgacgtcaatgggtggagtatttacggtaaactgcccacttggcagtacatcaagtgtatcatatgccaagtacgccccctattgacgtcaatgacggtaaatggcccgcctggcattatgcccagtacatgaccttatgggactttcctacttggcagtacatctacgtattagtcatcgctattaccatggtgatgcggttttggcagtacatcaatgggcgtggatagcggtttgactcacggggatttccaagtctccaccccattgacgtcaatgggagtttgttttggcaccaaaatcaacgggactttccaaaatgtcgtaacaactccgccccattgacgcaaatgggcggtaggcgtgtacggtgggaggtctatataagcagagctctctggctaactagagaacccactgcttactggcttatcgaaattaatacgactcactatagggagacccaagctggctagcgtttaaacttaagcttggtaccgccaccatggaatccgatgagtctggcctgcccgccatggaaatcgagtgcagaatcaccggcaccctgaacggcgtggaatttgagctcgtgggcggaggcgagggcacacctgaacagggcagaatgaccaacaagatgaagtccaccaagggggccctgaccttcagcccctacctgctgtctcacgtgatgggctacggcttctaccacttcggcacctaccccagcggctacgagaaccctttcctgcacgccatcaacaacggcggctacaccaacacccggatcgagaagtacgaggacggcggcgtgctgcacgtgtccttcagctacagatacgaggccggcagagtgatcggcgacttcaaagtgatgggcaccggattccccgaggacagcgtgatcttcaccgacaagatcatccggtccaacgccaccgtggaacatctgcaccccatgggcgacaacgacctggacggcagcttcaccagaaccttctccctgcgggatggcggctactacagcagcgtggtggacagccacatgcacttcaagagcgccatccaccccagcatcctccagaacggcggacccatgttcgccttcagacgggtggaagaggaccacagcaacaccgagctgggcatcgtggaataccagcacgccttcaagacccccgatgccgatgccggcgaggaatgagtcgagtctagagggcccgtttaaacccgctgatcagcctcgactgtgccttctagttgccagccatctgttgtttgcccctcccccgtgccttccttgaccctggaaggtgccactcccactgtcctttcctaataaaatgaggaaattgcatcgcattgtctgagtaggtgtcattctattctggggggtggggtggggcaggacagcaagggggaggattgggaagacaatagcaggcatgctggggatgcggtgggctctatggcttctgaggcggaaagaaccagctggggctctagggggtatccccacgcgccctgtagcggcgcattaagcgcggcgggtgtggtggttacgcgcagcgtgaccgctacacttgccagcgccctagcgcccgctcctttcgctttcttcccttcctttctcgccacgttcgccggctttccccgtcaagctctaaatcgggggctccctttagggttccgatttagtgctttacggcacctcgaccccaaaaaacttgattagggtgatggttcacgtagtgggccatcgccctgatagacggtttttcgccctttgacgttggagtccacgttctttaatagtggactcttgttccaaactggaacaacactcaaccctatctcggtctattcttttgatttataagggattttgccgatttcggcctattggttaaaaaatgagctgatttaacaaaaatttaacgcgaattaattctgtggaatgtgtgtcagttagggtgtggaaagtccccaggctccccagcaggcagaagtatgcaaagcatgcatctcaattagtcagcaaccaggtgtggaaagtccccaggctccccagcaggcagaagtatgcaaagcatgcatctcaattagtcagcaaccatagtcccgcccctaactccgcccatcccgcccctaactccgcccagttccgcccattctccgccccatggctgactaattttttttatttatgcagaggccgaggccgcctctgcctctgagctattccagaagtagtgaggaggcttttttggaggcctaggcttttgcaaaaagctcccgggagcttgtatatccattttcggatctgatcaagagacaggatgaggatcgtttcgcatgattgaacaagatggattgcacgcaggttctccggccgcttgggtggagaggctattcggctatgactgggcacaacagacaatcggctgctctgatgccgccgtgttccggctgtcagcgcaggggcgcccggttctttttgtcaagaccgacctgtccggtgccctgaatgaactgcaggacgaggcagcgcggctatcgtggctggccacgacgggcgttccttgcgcagctgtgctcgacgttgtcactgaagcgggaagggactggctgctattgggcgaagtgccggggcaggatctcctgtcatctcaccttgctcctgccgagaaagtatccatcatggctgatgcaatgcggcggctgcatacgcttgatccggctacctgcccattcgaccaccaagcgaaacatcgcatcgagcgagcacgtactcggatggaagccggtcttgtcgatcaggatgatctggacgaagagcatcaggggctcgcgccagccgaactgttcgccaggctcaaggcgcgcatgcccgacggcgaggatctcgtcgtgacccatggcgatgcctgcttgccgaatatcatggtggaaaatggccgcttttctggattcatcgactgtggccggctgggtgtggcggaccgctatcaggacatagcgttggctacccgtgatattgctgaagagcttggcggcgaatgggctgaccgcttcctcgtgctttacggtatcgccgctcccgattcgcagcgcatcgccttctatcgccttcttgacgagttcttctgagcgggactctggggttcgaaatgaccgaccaagcgacgcccaacctgccatcacgagatttcgattccaccgccgccttctatgaaaggttgggcttcggaatcgttttccgggacgccggctggatgatcctccagcgcggggatctcatgctggagttcttcgcccaccccaacttgtttattgcagcttataatggttacaaataaagcaatagcatcacaaatttcacaaataaagcatttttttcactgcattctagttgtggtttgtccaaactcatcaatgtatcttatcatgtctgtataccgtcgacctctagctagagcttggcgtaatcatggtcatagctgtttcctgtgtgaaattgttatccgctcacaattccacacaacatacgagccggaagcataaagtgtaaagcctggggtgcctaatgagtgagctaactcacattaattgcgttgcgctcactgcccgctttccagtcgggaaacctgtcgtgccagctgcattaatgaatcggccaacgcgcggggagaggcggtttgcgtattgggcgctcttccgcttcctcgctcactgactcgctgcgctcggtcgttcggctgcggcgagcggtatcagctcactcaaaggcggtaatacggttatccacagaatcaggggataacgcaggaaagaacatgtgagcaaaaggccagcaaaaggccaggaaccgtaaaaaggccgcgttgctggcgtttttccataggctccgcccccctgacgagcatcacaaaaatcgacgctcaagtcagaggtggcgaaacccgacaggactataaagataccaggcgtttccccctggaagctccctcgtgcgctctcctgttccgaccctgccgcttaccggatacctgtccgcctttctcccttcgggaagcgtggcgctttctcatagctcacgctgtaggtatctcagttcggtgtaggtcgttcgctccaagctgggctgtgtgcacgaaccccccgttcagcccgaccgctgcgccttatccggtaactatcgtcttgagtccaacccggtaagacacgacttatcgccactggcagcagccactggtaacaggattagcagagcgaggtatgtaggcggtgctacagagttcttgaagtggtggcctaactacggctacactagaagaacagtatttggtatctgcgctctgctgaagccagttaccttcggaaaaagagttggtagctcttgatccggcaaacaaaccaccgctggtagcggtttttttgtttgcaagcagcagattacgcgcagaaaaaaaggatctcaagaagatcctttgatcttttctacggggtctgacgctcagtggaacgaaaactcacgttaagggattttggtcatgagattatcaaaaaggatcttcacctagatccttttaaattaaaaatgaagttttaaatcaatctaaagtatatatgagtaaacttggtctgacagttaccaatgcttaatcagtgaggcacctatctcagcgatctgtctatttcgttcatccatagttgcctgactccccgtcgtgtagataactacgatacgggagggcttaccatctggccccagtgctgcaatgataccgcgagacccacgctcaccggctccagatttatcagcaataaaccagccagccggaagggccgagcgcagaagtggtcctgcaactttatccgcctccatccagtctattaattgttgccgggaagctagagtaagtagttcgccagttaatagtttgcgcaacgttgttgccattgctacaggcatcgtggtgtcacgctcgtcgtttggtatggcttcattcagctccggttcccaacgatcaaggcgagttacatgatcccccatgttgtgcaaaaaagcggttagctccttcggtcctccgatcgttgtcagaagtaagttggccgcagtgttatcactcatggttatggcagcactgcataattctcttactgtcatgccatccgtaagatgcttttctgtgactggtgagtactcaaccaagtcattctgagaatagtgtatgcggcgaccgagttgctcttgcccggcgtcaatacgggataataccgcgccacatagcagaactttaaaagtgctcatcattggaaaacgttcttcggggcgaaaactctcaaggatcttaccgctgttgagatccagttcgatgtaacccactcgtgcacccaactgatcttcagcatcttttactttcaccagcgtttctgggtgagcaaaaacaggaaggcaaaatgccgcaaaaaagggaataagggcgacacggaaatgttgaatactcatactcttcctttttcaatattattgaagcatttatcagggttattgtctcatgagcggatacatatttgaatgtatttagaaaaataaacaaataggggttccgcgcacatttccccgaaaagtgccacctgacgtc

SEQ ID NO: 6 - DNA, 6068 bp, Artificial Sequence
  pcDNA3.1_RFP vector V1.A.6
gacggatcgggagatctcccgatcccctatggtgcactctcagtacaatctgctctgatgccgcatagttaagccagtatctgctccctgcttgtgtgttggaggtcgctgagtagtgcgcgagcaaaatttaagctacaacaaggcaaggcttgaccgacaattgcatgaagaatctgcttagggttaggcgttttgcgctgcttcgcgatgtacgggccagatatacgcgttgacattgattattgactagttattaatagtaatcaattacggggtcattagttcatagcccatatatggagttccgcgttacataacttacggtaaatggcccgcctggctgaccgcccaacgacccccgcccattgacgtcaataatgacgtatgttcccatagtaacgccaatagggactttccattgacgtcaatgggtggagtatttacggtaaactgcccacttggcagtacatcaagtgtatcatatgccaagtacgccccctattgacgtcaatgacggtaaatggcccgcctggcattatgcccagtacatgaccttatgggactttcctacttggcagtacatctacgtattagtcatcgctattaccatggtgatgcggttttggcagtacatcaatgggcgtggatagcggtttgactcacggggatttccaagtctccaccccattgacgtcaatgggagtttgttttggcaccaaaatcaacgggactttccaaaatgtcgtaacaactccgccccattgacgcaaatgggcggtaggcgtgtacggtgggaggtctatataagcagagctctctggctaactagagaacccactgcttactggcttatcgaaattaatacgactcactatagggagacccaagctggctagcgtttaaacttaagcttggtaccgccaccatgagcgagctgatcaaagaaaacatgcacatgaagctgtacatggaaggcaccgtgaacaaccaccacttcaagtgcaccagcgagggcgagggcaagccttacgagggcacccagaccatgaagatcaaggtggtggaaggcggccctctgcccttcgcctttgatatcctggccaccagctttatgtacggcagcaaggccttcatcaaccacacccagggcatccccgatttcttcaagcagagcttccccgagggcttcacctgggagcggatcaccacatacgaggacggcggagtgctgaccgccacccaggataccagcttccagaacggctgcatcatctacaacgtgaagattaacggcgtgaacttccccagcaacggccccgtgatgcagaagaaaaccagaggctgggaggccaacaccgagatgctgtaccctgccgatggcggcctgagaggccattctcagatggccctgaaactcgtgggcggaggctacctgcactgctccttcaagaccacctacagaagcaagaagcccgccaagaacctgaagatgcccggcttccacttcgtggaccaccggctggaacggatcaaagaggccgacaaagaaacctacgtggaacagcacgagatggccgtggccaagtactgcgacctgcctagcaagctgggccacagatgagtcgagtctagagggcccgtttaaacccgctgatcagcctcgactgtgccttctagttgccagccatctgttgtttgcccctcccccgtgccttccttgaccctggaaggtgccactcccactgtcctttcctaataaaatgaggaaattgcatcgcattgtctgagtaggtgtcattctattctggggggtggggtggggcaggacagcaagggggaggattgggaagacaatagcaggcatgctggggatgcggtgggctctatggcttctgaggcggaaagaaccagctggggctctagggggtatccccacgcgccctgtagcggcgcattaagcgcggcgggtgtggtggttacgcgcagcgtgaccgctacacttgccagcgccctagcgcccgctcctttcgctttcttcccttcctttctcgccacgttcgccggctttccccgtcaagctctaaatcgggggctccctttagggttccgatttagtgctttacggcacctcgaccccaaaaaacttgattagggtgatggttcacgtagtgggccatcgccctgatagacggtttttcgccctttgacgttggagtccacgttctttaatagtggactcttgttccaaactggaacaacactcaaccctatctcggtctattcttttgatttataagggattttgccgatttcggcctattggttaaaaaatgagctgatttaacaaaaatttaacgcgaattaattctgtggaatgtgtgtcagttagggtgtggaaagtccccaggctccccagcaggcagaagtatgcaaagcatgcatctcaattagtcagcaaccaggtgtggaaagtccccaggctccccagcaggcagaagtatgcaaagcatgcatctcaattagtcagcaaccatagtcccgcccctaactccgcccatcccgcccctaactccgcccagttccgcccattctccgccccatggctgactaattttttttatttatgcagaggccgaggccgcctctgcctctgagctattccagaagtagtgaggaggcttttttggaggcctaggcttttgcaaaaagctcccgggagcttgtatatccattttcggatctgatcaagagacaggatgaggatcgtttcgcatgattgaacaagatggattgcacgcaggttctccggccgcttgggtggagaggctattcggctatgactgggcacaacagacaatcggctgctctgatgccgccgtgttccggctgtcagcgcaggggcgcccggttctttttgtcaagaccgacctgtccggtgccctgaatgaactgcaggacgaggcagcgcggctatcgtggctggccacgacgggcgttccttgcgcagctgtgctcgacgttgtcactgaagcgggaagggactggctgctattgggcgaagtgccggggcaggatctcctgtcatctcaccttgctcctgccgagaaagtatccatcatggctgatgcaatgcggcggctgcatacgcttgatccggctacctgcccattcgaccaccaagcgaaacatcgcatcgagcgagcacgtactcggatggaagccggtcttgtcgatcaggatgatctggacgaagagcatcaggggctcgcgccagccgaactgttcgccaggctcaaggcgcgcatgcccgacggcgaggatctcgtcgtgacccatggcgatgcctgcttgccgaatatcatggtggaaaatggccgcttttctggattcatcgactgtggccggctgggtgtggcggaccgctatcaggacatagcgttggctacccgtgatattgctgaagagcttggcggcgaatgggctgaccgcttcctcgtgctttacggtatcgccgctcccgattcgcagcgcatcgccttctatcgccttcttgacgagttcttctgagcgggactctggggttcgaaatgaccgaccaagcgacgcccaacctgccatcacgagatttcgattccaccgccgccttctatgaaaggttgggcttcggaatcgttttccgggacgccggctggatgatcctccagcgcggggatctcatgctggagttcttcgcccaccccaacttgtttattgcagcttataatggttacaaataaagcaatagcatcacaaatttcacaaataaagcatttttttcactgcattctagttgtggtttgtccaaactcatcaatgtatcttatcatgtctgtataccgtcgacctctagctagagcttggcgtaatcatggtcatagctgtttcctgtgtgaaattgttatccgctcacaattccacacaacatacgagccggaagcataaagtgtaaagcctggggtgcctaatgagtgagctaactcacattaattgcgttgcgctcactgcccgctttccagtcgggaaacctgtcgtgccagctgcattaatgaatcggccaacgcgcggggagaggcggtttgcgtattgggcgctcttccgcttcctcgctcactgactcgctgcgctcggtcgttcggctgcggcgagcggtatcagctcactcaaaggcggtaatacggttatccacagaatcaggggataacgcaggaaagaacatgtgagcaaaaggccagcaaaaggccaggaaccgtaaaaaggccgcgttgctggcgtttttccataggctccgcccccctgacgagcatcacaaaaatcgacgctcaagtcagaggtggcgaaacccgacaggactataaagataccaggcgtttccccctggaagctccctcgtgcgctctcctgttccgaccctgccgcttaccggatacctgtccgcctttctcccttcgggaagcgtggcgctttctcatagctcacgctgtaggtatctcagttcggtgtaggtcgttcgctccaagctgggctgtgtgcacgaaccccccgttcagcccgaccgctgcgccttatccggtaactatcgtcttgagtccaacccggtaagacacgacttatcgccactggcagcagccactggtaacaggattagcagagcgaggtatgtaggcggtgctacagagttcttgaagtggtggcctaactacggctacactagaagaacagtatttggtatctgcgctctgctgaagccagttaccttcggaaaaagagttggtagctcttgatccggcaaacaaaccaccgctggtagcggtttttttgtttgcaagcagcagattacgcgcagaaaaaaaggatctcaagaagatcctttgatcttttctacggggtctgacgctcagtggaacgaaaactcacgttaagggattttggtcatgagattatcaaaaaggatcttcacctagatccttttaaattaaaaatgaagttttaaatcaatctaaagtatatatgagtaaacttggtctgacagttaccaatgcttaatcagtgaggcacctatctcagcgatctgtctatttcgttcatccatagttgcctgactccccgtcgtgtagataactacgatacgggagggcttaccatctggccccagtgctgcaatgataccgcgagacccacgctcaccggctccagatttatcagcaataaaccagccagccggaagggccgagcgcagaagtggtcctgcaactttatccgcctccatccagtctattaattgttgccgggaagctagagtaagtagttcgccagttaatagtttgcgcaacgttgttgccattgctacaggcatcgtggtgtcacgctcgtcgtttggtatggcttcattcagctccggttcccaacgatcaaggcgagttacatgatcccccatgttgtgcaaaaaagcggttagctccttcggtcctccgatcgttgtcagaagtaagttggccgcagtgttatcactcatggttatggcagcactgcataattctcttactgtcatgccatccgtaagatgcttttctgtgactggtgagtactcaaccaagtcattctgagaatagtgtatgcggcgaccgagttgctcttgcccggcgtcaatacgggataataccgcgccacatagcagaactttaaaagtgctcatcattggaaaacgttcttcggggcgaaaactctcaaggatcttaccgctgttgagatccagttcgatgtaacccactcgtgcacccaactgatcttcagcatcttttactttcaccagcgtttctgggtgagcaaaaacaggaaggcaaaatgccgcaaaaaagggaataagggcgacacggaaatgttgaatactcatactcttcctttttcaatattattgaagcatttatcagggttattgtctcatgagcggatacatatttgaatgtatttagaaaaataaacaaataggggttccgcgcacatttccccgaaaagtgccacctgacgtc

SEQ ID NO: 7 - DNA, 2508 bp, Artificial Sequence
  pMA-SV40pA vector V1.C.2
ctaaattgtaagcgttaatattttgttaaaattcgcgttaaatttttgttaaatcagctcattttttaaccaataggccgaaatcggcaaaatcccttataaatcaaaagaatagaccgagatagggttgagtggccgctacagggcgctcccattcgccattcaggctgcgcaactgttgggaagggcgtttcggtgcgggcctcttcgctattacgccagctggcgaaagggggatgtgctgcaaggcgattaagttgggtaacgccagggttttcccagtcacgacgttgtaaaacgacggccagtgagcgcgacgtaatacgactcactatagggcgaattggcggaaggccgtcaaggccgcatgaattgttgttgttaacttgtttattgcagcttataatggttacaaataaagcaatagcatcacaaatttcacaaataaagcatttttttcactgcattctagttgtggtttgtccaaactcatcaatgtatcttatcatgtctggatctgcggatccaatctcgagctgggcctcatgggccttccgctcactgcccgctttccagtcgggaaacctgtcgtgccagctgcattaacatggtcatagctgtttccttgcgtattgggcgctctccgcttcctcgctcactgactcgctgcgctcggtcgttcgggtaaagcctggggtgcctaatgagcaaaaggccagcaaaaggccaggaaccgtaaaaaggccgcgttgctggcgtttttccataggctccgcccccctgacgagcatcacaaaaatcgacgctcaagtcagaggtggcgaaacccgacaggactataaagataccaggcgtttccccctggaagctccctcgtgcgctctcctgttccgaccctgccgcttaccggatacctgtccgcctttctcccttcgggaagcgtggcgctttctcatagctcacgctgtaggtatctcagttcggtgtaggtcgttcgctccaagctgggctgtgtgcacgaaccccccgttcagcccgaccgctgcgccttatccggtaactatcgtcttgagtccaacccggtaagacacgacttatcgccactggcagcagccactggtaacaggattagcagagcgaggtatgtaggcggtgctacagagttcttgaagtggtggcctaactacggctacactagaagaacagtatttggtatctgcgctctgctgaagccagttaccttcggaaaaagagttggtagctcttgatccggcaaacaaaccaccgctggtagcggtggtttttttgtttgcaagcagcagattacgcgcagaaaaaaaggatctcaagaagatcctttgatcttttctacggggtctgacgctcagtggaacgaaaactcacgttaagggattttggtcatgagattatcaaaaaggatcttcacctagatccttttaaattaaaaatgaagttttaaatcaatctaaagtatatatgagtaaacttggtctgacagttaccaatgcttaatcagtgaggcacctatctcagcgatctgtctatttcgttcatccatagttgcctgactccccgtcgtgtagataactacgatacgggagggcttaccatctggccccagtgctgcaatgataccgcgagaaccacgctcaccggctccagatttatcagcaataaaccagccagccggaagggccgagcgcagaagtggtcctgcaactttatccgcctccatccagtctattaattgttgccgggaagctagagtaagtagttcgccagttaatagtttgcgcaacgttgttgccattgctacaggcatcgtggtgtcacgctcgtcgtttggtatggcttcattcagctccggttcccaacgatcaaggcgagttacatgatcccccatgttgtgcaaaaaagcggttagctccttcggtcctccgatcgttgtcagaagtaagttggccgcagtgttatcactcatggttatggcagcactgcataattctcttactgtcatgccatccgtaagatgcttttctgtgactggtgagtactcaaccaagtcattctgagaatagtgtatgcggcgaccgagttgctcttgcccggcgtcaatacgggataataccgcgccacatagcagaactttaaaagtgctcatcattggaaaacgttcttcggggcgaaaactctcaaggatcttaccgctgttgagatccagttcgatgtaacccactcgtgcacccaactgatcttcagcatcttttactttcaccagcgtttctgggtgagcaaaaacaggaaggcaaaatgccgcaaaaaagggaataagggcgacacggaaatgttgaatactcatactcttcctttttcaatattattgaagcatttatcagggttattgtctcatgagcggatacatatttgaatgtatttagaaaaataaacaaataggggttccgcgcacatttccccgaaaagtgccac

SEQ ID NO: 8 - DNA, 6275 bp, Artificial Sequence
  pMA-CS-JG9-TCRbeta vector V3.C.5
gacggatcgggagatctcccgatcccctatggtgcactctcagtacaatctgctctgatgccgcatagttaagccagtatctgctccctgcttgtgtgttggaggtcgctgagtagtgcgcgagcaaaatttaagctacaacaaggcaaggcttgaccgacaattgcatgaagaatctgcttagggttaggcgttttgcgctgcttcgcgatgtacgggccagatatacgcgttgacattgattattgactagttattaatagtaatcaattacggggtcattagttcatagcccatatatggagttccgcgttacataacttacggtaaatggcccgcctggctgaccgcccaacgacccccgcccattgacgtcaataatgacgtatgttcccatagtaacgccaatagggactttccattgacgtcaatgggtggagtatttacggtaaactgcccacttggcagtacatcaagtgtatcatatgccaagtacgccccctattgacgtcaatgacggtaaatggcccgcctggcattatgcccagtacatgaccttatgggactttcctacttggcagtacatctacgtattagtcatcgctattaccatggtgatgcggttttggcagtacatcaatgggcgtggatagcggtttgactcacggggatttccaagtctccaccccattgacgtcaatgggagtttgttttggcaccaaaatcaacgggactttccaaaatgtcgtaacaactccgccccattgacgcaaatgggcggtaggcgtgtacggtgggaggtctatataagcagagctctctggctaactagagaacccactgcttactggcttatcgaaattaatacgactcactatagggagacccaagctggctagcgtttaaacttaagcttggtaccgagctcggatccaccatggactcctggaccttctgctgtgtgtccctttgcatcctggtagcaaagcacacagatgctggagttatccagtcaccccggcacgaggtgacagagatgggacaagaagtgactctgagatgtaaaccaatttcaggacacgactaccttttctggtacagacagaccatgatgcggggactggagttgctcatttactttaacaacaacgttccgatagatgattcagggatgcccgaggatcgattctcagctaagatgcctaatgcatcattctccactctgaagatccagccctcagaacccagggactcagctgtgtacttctgtgccagcagttcggcaaactatggctacaccttcggttcggggaccaggttaaccgttgtagaggacctgaacaaggtgttcccacccgaggtcgctgtgtttgagccatcagaagcagagatctcccacacccaaaaggccacactggtgtgcctggccacaggcttcttccctgaccacgtggagctgagctggtgggtgaatgggaaggaggtgcacagtggggtcagcacggacccgcagcccctcaaggagcagcccgccctcaatgactccagatactgcctgagcagccgcctgagggtctcggccaccttctggcagaacccccgcaaccacttccgctgtcaagtccagttctacgggctctcggagaatgacgagtggacccaggatagggccaaacccgtcacccagatcgtcagcgccgaggcctggggtagagcagactgtggctttacctcggtgtcctaccagcaaggggtcctgtctgccaccatcctctatgagatcctgctagggaaggccaccctgtatgctgtgctggtcagcgcccttgtgttgatggccatggtcaagagaaaggatttctgattctagacgactgtgccttctagttgccagccatctgttgtttgcccctcccccgtgccttccttgaccctggaaggtgccactcccactgtcctttcctaataaaatgaggaaattgcatcgcattgtctgagtaggtgtcattctattctggggggtggggtggggcaggacagcaagggggaggattgggaagacaatagcaggcatgctggggatgcggtgggctctatggcttctgaggcggaaagaaccagctggggctctagggggtatccccacgcgccctgtagcggcgcattaagcgcggcgggtgtggtggttacgcgcagcgtgaccgctacacttgccagcgccctagcgcccgctcctttcgctttcttcccttcctttctcgccacgttcgccggctttccccgtcaagctctaaatcgggggctccctttagggttccgatttagtgctttacggcacctcgaccccaaaaaacttgattagggtgatggttcacgtagtgggccatcgccctgatagacggtttttcgccctttgacgttggagtccacgttctttaatagtggactcttgttccaaactggaacaacactcaaccctatctcggtctattcttttgatttataagggattttgccgatttcggcctattggttaaaaaatgagctgatttaacaaaaatttaacgcgaattaattctgtggaatgtgtgtcagttagggtgtggaaagtccccaggctccccagcaggcagaagtatgcaaagcatgcatctcaattagtcagcaaccaggtgtggaaagtccccaggctccccagcaggcagaagtatgcaaagcatgcatctcaattagtcagcaaccatagtcccgcccctaactccgcccatcccgcccctaactccgcccagttccgcccattctccgccccatggctgactaattttttttatttatgcagaggccgaggccgcctctgcctctgagctattccagaagtagtgaggaggcttttttggaggcctaggcttttgcaaaaagctcccgggagcttgtatatccattttcggatctgatcaagagacaggatgaggatcgtttcgcatgattgaacaagatggattgcacgcaggttctccggccgcttgggtggagaggctattcggctatgactgggcacaacagacaatcggctgctctgatgccgccgtgttccggctgtcagcgcaggggcgcccggttctttttgtcaagaccgacctgtccggtgccctgaatgaactgcaggacgaggcagcgcggctatcgtggctggccacgacgggcgttccttgcgcagctgtgctcgacgttgtcactgaagcgggaagggactggctgctattgggcgaagtgccggggcaggatctcctgtcatctcaccttgctcctgccgagaaagtatccatcatggctgatgcaatgcggcggctgcatacgcttgatccggctacctgcccattcgaccaccaagcgaaacatcgcatcgagcgagcacgtactcggatggaagccggtcttgtcgatcaggatgatctggacgaagagcatcaggggctcgcgccagccgaactgttcgccaggctcaaggcgcgcatgcccgacggcgaggatctcgtcgtgacccatggcgatgcctgcttgccgaatatcatggtggaaaatggccgcttttctggattcatcgactgtggccggctgggtgtggcggaccgctatcaggacatagcgttggctacccgtgatattgctgaagagcttggcggcgaatgggctgaccgcttcctcgtgctttacggtatcgccgctcccgattcgcagcgcatcgccttctatcgccttcttgacgagttcttctgagcgggactctggggttcgaaatgaccgaccaagcgacgcccaacctgccatcacgagatttcgattccaccgccgccttctatgaaaggttgggcttcggaatcgttttccgggacgccggctggatgatcctccagcgcggggatctcatgctggagttcttcgcccaccccaacttgtttattgcagcttataatggttacaaataaagcaatagcatcacaaatttcacaaataaagcatttttttcactgcattctagttgtggtttgtccaaactcatcaatgtatcttatcatgtctgtataccgtcgacctctagctagagcttggcgtaatcatggtcatagctgtttcctgtgtgaaattgttatccgctcacaattccacacaacatacgagccggaagcataaagtgtaaagcctggggtgcctaatgagtgagctaactcacattaattgcgttgcgctcactgcccgctttccagtcgggaaacctgtcgtgccagctgcattaatgaatcggccaacgcgcggggagaggcggtttgcgtattgggcgctcttccgcttcctcgctcactgactcgctgcgctcggtcgttcggctgcggcgagcggtatcagctcactcaaaggcggtaatacggttatccacagaatcaggggataacgcaggaaagaacatgtgagcaaaaggccagcaaaaggccaggaaccgtaaaaaggccgcgttgctggcgtttttccataggctccgcccccctgacgagcatcacaaaaatcgacgctcaagtcagaggtggcgaaacccgacaggactataaagataccaggcgtttccccctggaagctccctcgtgcgctctcctgttccgaccctgccgcttaccggatacctgtccgcctttctcccttcgggaagcgtggcgctttctcatagctcacgctgtaggtatctcagttcggtgtaggtcgttcgctccaagctgggctgtgtgcacgaaccccccgttcagcccgaccgctgcgccttatccggtaactatcgtcttgagtccaacccggtaagacacgacttatcgccactggcagcagccactggtaacaggattagcagagcgaggtatgtaggcggtgctacagagttcttgaagtggtggcctaactacggctacactagaagaacagtatttggtatctgcgctctgctgaagccagttaccttcggaaaaagagttggtagctcttgatccggcaaacaaaccaccgctggtagcggtttttttgtttgcaagcagcagattacgcgcagaaaaaaaggatctcaagaagatcctttgatcttttctacggggtctgacgctcagtggaacgaaaactcacgttaagggattttggtcatgagattatcaaaaaggatcttcacctagatccttttaaattaaaaatgaagttttaaatcaatctaaagtatatatgagtaaacttggtctgacagttaccaatgcttaatcagtgaggcacctatctcagcgatctgtctatttcgttcatccatagttgcctgactccccgtcgtgtagataactacgatacgggagggcttaccatctggccccagtgctgcaatgataccgcgagacccacgctcaccggctccagatttatcagcaataaaccagccagccggaagggccgagcgcagaagtggtcctgcaactttatccgcctccatccagtctattaattgttgccgggaagctagagtaagtagttcgccagttaatagtttgcgcaacgttgttgccattgctacaggcatcgtggtgtcacgctcgtcgtttggtatggcttcattcagctccggttcccaacgatcaaggcgagttacatgatcccccatgttgtgcaaaaaagcggttagctccttcggtcctccgatcgttgtcagaagtaagttggccgcagtgttatcactcatggttatggcagcactgcataattctcttactgtcatgccatccgtaagatgcttttctgtgactggtgagtactcaaccaagtcattctgagaatagtgtatgcggcgaccgagttgctcttgcccggcgtcaatacgggataataccgcgccacatagcagaactttaaaagtgctcatcattggaaaacgttcttcggggcgaaaactctcaaggatcttaccgctgttgagatccagttcgatgtaacccactcgtgcacccaactgatcttcagcatcttttactttcaccagcgtttctgggtgagcaaaaacaggaaggcaaaatgccgcaaaaaagggaataagggcgacacggaaatgttgaatactcatactcttcctttttcaatattattgaagcatttatcagggttattgtctcatgagcggatacatatttgaatgtatttagaaaaataaacaaataggggttccgcgcacatttccccgaaaagtgccacctgacgtc

SEQ ID NO: 9 - DNA, 3182 bp, Artificial Sequence
  pMA-F14-GFP-F15 vector V4.H9
ctaaattgtaagcgttaatattttgttaaaattcgcgttaaatttttgttaaatcagctcattttttaaccaataggccgaaatcggcaaaatcccttataaatcaaaagaatagaccgagatagggttgagtggccgctacagggcgctcccattcgccattcaggctgcgcaactgttgggaagggcgtttcggtgcgggcctcttcgctattacgccagctggcgaaagggggatgtgctgcaaggcgattaagttgggtaacgccagggttttcccagtcacgacgttgtaaaacgacggccagtgagcgcgacgtaatacgactcactatagggcgaattggcggaaggccgtcaaggccgcatgaattcgctaccgggaagttcctattccgaagttcctattctatcagaagtataggaacttcaggtaccgccaccatggaatccgatgagtctggcctgcccgccatggaaatcgagtgcagaatcaccggcaccctgaacggcgtggaatttgagctcgtgggcggaggcgagggcacacctgaacagggcagaatgaccaacaagatgaagtccaccaagggggccctgaccttcagcccctacctgctgtctcacgtgatgggctacggcttctaccacttcggcacctaccccagcggctacgagaaccctttcctgcacgccatcaacaacggcggctacaccaacacccggatcgagaagtacgaggacggcggcgtgctgcacgtgtccttcagctacagatacgaggccggcagagtgatcggcgacttcaaagtgatgggcaccggattccccgaggacagcgtgatcttcaccgacaagatcatccggtccaacgccaccgtggaacatctgcaccccatgggcgacaacgacctggacggcagcttcaccagaaccttctccctgcgggatggcggctactacagcagcgtggtggacagccacatgcacttcaagagcgccatccaccccagcatcctccagaacggcggacccatgttcgccttcagacgggtggaagaggaccacagcaacaccgagctgggcatcgtggaataccagcacgccttcaagacccccgatgccgatgccggcgaggaatgagtcgagtctagacgaagttcctattccgaagttcctattcttataggagtataggaacttcctcgagctgggcctcatgggccttccgctcactgcccgctttccagtcgggaaacctgtcgtgccagctgcattaacatggtcatagctgtttccttgcgtattgggcgctctccgcttcctcgctcactgactcgctgcgctcggtcgttcgggtaaagcctggggtgcctaatgagcaaaaggccagcaaaaggccaggaaccgtaaaaaggccgcgttgctggcgtttttccataggctccgcccccctgacgagcatcacaaaaatcgacgctcaagtcagaggtggcgaaacccgacaggactataaagataccaggcgtttccccctggaagctccctcgtgcgctctcctgttccgaccctgccgcttaccggatacctgtccgcctttctcccttcgggaagcgtggcgctttctcatagctcacgctgtaggtatctcagttcggtgtaggtcgttcgctccaagctgggctgtgtgcacgaaccccccgttcagcccgaccgctgcgccttatccggtaactatcgtcttgagtccaacccggtaagacacgacttatcgccactggcagcagccactggtaacaggattagcagagcgaggtatgtaggcggtgctacagagttcttgaagtggtggcctaactacggctacactagaagaacagtatttggtatctgcgctctgctgaagccagttaccttcggaaaaagagttggtagctcttgatccggcaaacaaaccaccgctggtagcggtggtttttttgtttgcaagcagcagattacgcgcagaaaaaaaggatctcaagaagatcctttgatcttttctacggggtctgacgctcagtggaacgaaaactcacgttaagggattttggtcatgagattatcaaaaaggatcttcacctagatccttttaaattaaaaatgaagttttaaatcaatctaaagtatatatgagtaaacttggtctgacagttaccaatgcttaatcagtgaggcacctatctcagcgatctgtctatttcgttcatccatagttgcctgactccccgtcgtgtagataactacgatacgggagggcttaccatctggccccagtgctgcaatgataccgcgagaaccacgctcaccggctccagatttatcagcaataaaccagccagccggaagggccgagcgcagaagtggtcctgcaactttatccgcctccatccagtctattaattgttgccgggaagctagagtaagtagttcgccagttaatagtttgcgcaacgttgttgccattgctacaggcatcgtggtgtcacgctcgtcgtttggtatggcttcattcagctccggttcccaacgatcaaggcgagttacatgatcccccatgttgtgcaaaaaagcggttagctccttcggtcctccgatcgttgtcagaagtaagttggccgcagtgttatcactcatggttatggcagcactgcataattctcttactgtcatgccatccgtaagatgcttttctgtgactggtgagtactcaaccaagtcattctgagaatagtgtatgcggcgaccgagttgctcttgcccggcgtcaatacgggataataccgcgccacatagcagaactttaaaagtgctcatcattggaaaacgttcttcggggcgaaaactctcaaggatcttaccgctgttgagatccagttcgatgtaacccactcgtgcacccaactgatcttcagcatcttttactttcaccagcgtttctgggtgagcaaaaacaggaaggcaaaatgccgcaaaaaagggaataagggcgacacggaaatgttgaatactcatactcttcctttttcaatattattgaagcatttatcagggttattgtctcatgagcggatacatatttgaatgtatttagaaaaataaacaaataggggttccgcgcacatttccccgaaaagtgccac

SEQ ID NO: 10 - DNA, 3291 bp, Artificial Sequence
  pMA-F14-TCR-JG9-alpha-F15 vector V7.A.3
acgaagttcctattccgaagttcctattcttataggagtataggaacttcctcgagctgggcctcatgggccttccgctcactgcccgctttccagtcgggaaacctgtcgtgccagctgcattaacatggtcatagctgtttccttgcgtattgggcgctctccgcttcctcgctcactgactcgctgcgctcggtcgttcgggtaaagcctggggtgcctaatgagcaaaaggccagcaaaaggccaggaaccgtaaaaaggccgcgttgctggcgtttttccataggctccgcccccctgacgagcatcacaaaaatcgacgctcaagtcagaggtggcgaaacccgacaggactataaagataccaggcgtttccccctggaagctccctcgtgcgctctcctgttccgaccctgccgcttaccggatacctgtccgcctttctcccttcgggaagcgtggcgctttctcatagctcacgctgtaggtatctcagttcggtgtaggtcgttcgctccaagctgggctgtgtgcacgaaccccccgttcagcccgaccgctgcgccttatccggtaactatcgtcttgagtccaacccggtaagacacgacttatcgccactggcagcagccactggtaacaggattagcagagcgaggtatgtaggcggtgctacagagttcttgaagtggtggcctaactacggctacactagaagaacagtatttggtatctgcgctctgctgaagccagttaccttcggaaaaagagttggtagctcttgatccggcaaacaaaccaccgctggtagcggtggtttttttgtttgcaagcagcagattacgcgcagaaaaaaaggatctcaagaagatcctttgatcttttctacggggtctgacgctcagtggaacgaaaactcacgttaagggattttggtcatgagattatcaaaaaggatcttcacctagatccttttaaattaaaaatgaagttttaaatcaatctaaagtatatatgagtaaacttggtctgacagttaccaatgcttaatcagtgaggcacctatctcagcgatctgtctatttcgttcatccatagttgcctgactccccgtcgtgtagataactacgatacgggagggcttaccatctggccccagtgctgcaatgataccgcgagaaccacgctcaccggctccagatttatcagcaataaaccagccagccggaagggccgagcgcagaagtggtcctgcaactttatccgcctccatccagtctattaattgttgccgggaagctagagtaagtagttcgccagttaatagtttgcgcaacgttgttgccattgctacaggcatcgtggtgtcacgctcgtcgtttggtatggcttcattcagctccggttcccaacgatcaaggcgagttacatgatcccccatgttgtgcaaaaaagcggttagctccttcggtcctccgatcgttgtcagaagtaagttggccgcagtgttatcactcatggttatggcagcactgcataattctcttactgtcatgccatccgtaagatgcttttctgtgactggtgagtactcaaccaagtcattctgagaatagtgtatgcggcgaccgagttgctcttgcccggcgtcaatacgggataataccgcgccacatagcagaactttaaaagtgctcatcattggaaaacgttcttcggggcgaaaactctcaaggatcttaccgctgttgagatccagttcgatgtaacccactcgtgcacccaactgatcttcagcatcttttactttcaccagcgtttctgggtgagcaaaaacaggaaggcaaaatgccgcaaaaaagggaataagggcgacacggaaatgttgaatactcatactcttcctttttcaatattattgaagcatttatcagggttattgtctcatgagcggatacatatttgaatgtatttagaaaaataaacaaataggggttccgcgcacatttccccgaaaagtgccacctaaattgtaagcgttaatattttgttaaaattcgcgttaaatttttgttaaatcagctcattttttaaccaataggccgaaatcggcaaaatcccttataaatcaaaagaatagaccgagatagggttgagtggccgctacagggcgctcccattcgccattcaggctgcgcaactgttgggaagggcgtttcggtgcgggcctcttcgctattacgccagctggcgaaagggggatgtgctgcaaggcgattaagttgggtaacgccagggttttcccagtcacgacgttgtaaaacgacggccagtgagcgcgacgtaatacgactcactatagggcgaattggcggaaggccgtcaaggccgcatgaattcgctaccgggaagttcctattccgaagttcctattctatcagaagtataggaacttcaggtacgccaccatgctccttgaacatttattaataatcttgtggatgcagctgacatgggtcagtggtcaacagctgaatcagagtcctcaatctatgtttatccaggaaggagaagatgtctccatgaactgcacttcttcaagcatatttaacacctggctatggtacaagcaggaacctggggaaggtcctgtcctcttgatagccttatataaggctggtgaattgacctcaaatggaaggctgactgctcagtttggtataaccagaaaggacagcttcctgaatatctcagcatccatacctagtgatgtaggcatctacttctgcgctggacccatgaaaacctcctacgacaaggtgatatttgggccagggacaagcttatcagtcattccaaatatccagaaccctgaccctgccgtgtaccagctgagagactctaaatccagtgacaagtctgtctgcctattcaccgattttgattctcaaacaaatgtgtcacaaagtaaggattctgatgtgtatatcacagacaaaactgtgctagacatgaggtctatggacttcaagagcaacagtgctgtggcctggagcaacaaatctgactttgcatgtgcaaacgccttcaacaacagcattattccagaggacaccttcttccccagcccagaaagttcctgtgatgtcaagctggtcgagaaaagctttgaaacagatacgaacctaaactttcaaaacctgtcagtgattgggttccgaatcctcctcctgaaagtggccgggtttaatctgctcatgacgctgcggctgtggtccagctgactag

SEQ ID NO: 11 - DNA, 3408 bp, Artificial Sequence
  pMA-FRT-TCR-JG9-beta-F3 vector V7.A.4
ctaaattgtaagcgttaatattttgttaaaattcgcgttaaatttttgttaaatcagctcattttttaaccaataggccgaaatcggcaaaatcccttataaatcaaaagaatagaccgagatagggttgagtggccgctacagggcgctcccattcgccattcaggctgcgcaactgttgggaagggcgtttcggtgcgggcctcttcgctattacgccagctggcgaaagggggatgtgctgcaaggcgattaagttgggtaacgccagggttttcccagtcacgacgttgtaaaacgacggccagtgagcgcgacgtaatacgactcactatagggcgaattggcggaaggccgtcaaggccgcatgaattcgctaccgggaagttcctattccgaagttcctattctctagaaagtataggaacttcaggtacgccaccatggactcctggaccctctgctgtgtgtccctttgcatcctggtagcaaagcacacagatgctggagttatccagtcaccccggcacgaggtgacagagatgggacaagaagtgactctgagatgtaaaccaatttcaggacacgactaccttttctggtacagacagaccatgatgcggggactggagttgctcatttactttaacaacaacgttccgatagatgattcagggatgcccgaggatcgattctcagctaagatgcctaatgcatcattctccactctgaagatccagccctcagaacccagggactcagctgtgtacttttgcgccagcagttccgcaaactatggctacacctttggttcggggaccaggttaaccgttgtagaggacctgaacaaggtgttcccacccgaggtcgctgtgtttgagccatcagaagcagagatctcccacacccaaaaggccacactggtatgcctggccacaggcttctaccccgaccacgtggagctgagctggtgggtgaatgggaaggaggtgcacagtggggtcagcacagacccgcagcccctcaaggagcagcccgccctcaatgactccagatactgcctgagcagccgcctgagggtgtcggccaccttctggcagaacccccgcaaccacttccgctgtcaagtccagttctacgggctctcggagaatgacgagtggacccaggatagggccaaacccgtcacccagatcgtcagcgccgaggcctggggtagagcagactgtggcttcacctccgagtcttaccagcaaggggtcctgtctgccaccatcctctatgagatcttgctagggaaggccaccttgtatgccgtgctggtcagtgccctcgtgctgatggccatggtcaagagaaaggattccagaggctagctagacgaagttcctattccgaagttcctattcttcaaatagtataggaacttcctcgagctgggcctcatgggccttccgctcactgcccgctttccagtcgggaaacctgtcgtgccagctgcattaacatggtcatagctgtttccttgcgtattgggcgctctccgcttcctcgctcactgactcgctgcgctcggtcgttcgggtaaagcctggggtgcctaatgagcaaaaggccagcaaaaggccaggaaccgtaaaaaggccgcgttgctggcgtttttccataggctccgcccccctgacgagcatcacaaaaatcgacgctcaagtcagaggtggcgaaacccgacaggactataaagataccaggcgtttccccctggaagctccctcgtgcgctctcctgttccgaccctgccgcttaccggatacctgtccgcctttctcccttcgggaagcgtggcgctttctcatagctcacgctgtaggtatctcagttcggtgtaggtcgttcgctccaagctgggctgtgtgcacgaaccccccgttcagcccgaccgctgcgccttatccggtaactatcgtcttgagtccaacccggtaagacacgacttatcgccactggcagcagccactggtaacaggattagcagagcgaggtatgtaggcggtgctacagagttcttgaagtggtggcctaactacggctacactagaagaacagtatttggtatctgcgctctgctgaagccagttaccttcggaaaaagagttggtagctcttgatccggcaaacaaaccaccgctggtagcggtggtttttttgtttgcaagcagcagattacgcgcagaaaaaaaggatctcaagaagatcctttgatcttttctacggggtctgacgctcagtggaacgaaaactcacgttaagggattttggtcatgagattatcaaaaaggatcttcacctagatccttttaaattaaaaatgaagttttaaatcaatctaaagtatatatgagtaaacttggtctgacagttaccaatgcttaatcagtgaggcacctatctcagcgatctgtctatttcgttcatccatagttgcctgactccccgtcgtgtagataactacgatacgggagggcttaccatctggccccagtgctgcaatgataccgcgagaaccacgctcaccggctccagatttatcagcaataaaccagccagccggaagggccgagcgcagaagtggtcctgcaactttatccgcctccatccagtctattaattgttgccgggaagctagagtaagtagttcgccagttaatagtttgcgcaacgttgttgccattgctacaggcatcgtggtgtcacgctcgtcgtttggtatggcttcattcagctccggttcccaacgatcaaggcgagttacatgatcccccatgttgtgcaaaaaagcggttagctccttcggtcctccgatcgttgtcagaagtaagttggccgcagtgttatcactcatggttatggcagcactgcataattctcttactgtcatgccatccgtaagatgcttttctgtgactggtgagtactcaaccaagtcattctgagaatagtgtatgcggcgaccgagttgctcttgcccggcgtcaatacgggataataccgcgccacatagcagaactttaaaagtgctcatcattggaaaacgttcttcggggcgaaaactctcaaggatcttaccgctgttgagatccagttcgatgtaacccactcgtgcacccaactgatcttcagcatcttttactttcaccagcgtttctgggtgagcaaaaacaggaaggcaaaatgccgcaaaaaagggaataagggcgacacggaaatgttgaatactcatactcttcctttttcaatattattgaagcatttatcagggttattgtctcatgagcggatacatatttgaatgtatttagaaaaataaacaaataggggttccgcgcacatttccccgaaaagtgccac

SEQ ID NO: 12 - DNA, 3291 bp, Artificial Sequence
  F14-TCRaF15 CDR3degen.64mix vector V8.F.8
  variation 2803: /replace="n"= "a", "g", "c", or "t"
  variation 2808: /replace="n"= "a", "g", "c", or "t"
  variation 2814: /replace="n"= "a", "g", "c", or "t"
acgaagttcctattccgaagttcctattcttataggagtataggaacttcctcgagctgggcctcatgggccttccgctcactgcccgctttccagtcgggaaacctgtcgtgccagctgcattaacatggtcatagctgtttccttgcgtattgggcgctctccgcttcctcgctcactgactcgctgcgctcggtcgttcgggtaaagcctggggtgcctaatgagcaaaaggccagcaaaaggccaggaaccgtaaaaaggccgcgttgctggcgtttttccataggctccgcccccctgacgagcatcacaaaaatcgacgctcaagtcagaggtggcgaaacccgacaggactataaagataccaggcgtttccccctggaagctccctcgtgcgctctcctgttccgaccctgccgcttaccggatacctgtccgcctttctcccttcgggaagcgtggcgctttctcatagctcacgctgtaggtatctcagttcggtgtaggtcgttcgctccaagctgggctgtgtgcacgaaccccccgttcagcccgaccgctgcgccttatccggtaactatcgtcttgagtccaacccggtaagacacgacttatcgccactggcagcagccactggtaacaggattagcagagcgaggtatgtaggcggtgctacagagttcttgaagtggtggcctaactacggctacactagaagaacagtatttggtatctgcgctctgctgaagccagttaccttcggaaaaagagttggtagctcttgatccggcaaacaaaccaccgctggtagcggtggtttttttgtttgcaagcagcagattacgcgcagaaaaaaaggatctcaagaagatcctttgatcttttctacggggtctgacgctcagtggaacgaaaactcacgttaagggattttggtcatgagattatcaaaaaggatcttcacctagatccttttaaattaaaaatgaagttttaaatcaatctaaagtatatatgagtaaacttggtctgacagttaccaatgcttaatcagtgaggcacctatctcagcgatctgtctatttcgttcatccatagttgcctgactccccgtcgtgtagataactacgatacgggagggcttaccatctggccccagtgctgcaatgataccgcgagaaccacgctcaccggctccagatttatcagcaataaaccagccagccggaagggccgagcgcagaagtggtcctgcaactttatccgcctccatccagtctattaattgttgccgggaagctagagtaagtagttcgccagttaatagtttgcgcaacgttgttgccattgctacaggcatcgtggtgtcacgctcgtcgtttggtatggcttcattcagctccggttcccaacgatcaaggcgagttacatgatcccccatgttgtgcaaaaaagcggttagctccttcggtcctccgatcgttgtcagaagtaagttggccgcagtgttatcactcatggttatggcagcactgcataattctcttactgtcatgccatccgtaagatgcttttctgtgactggtgagtactcaaccaagtcattctgagaatagtgtatgcggcgaccgagttgctcttgcccggcgtcaatacgggataataccgcgccacatagcagaactttaaaagtgctcatcattggaaaacgttcttcggggcgaaaactctcaaggatcttaccgctgttgagatccagttcgatgtaacccactcgtgcacccaactgatcttcagcatcttttactttcaccagcgtttctgggtgagcaaaaacaggaaggcaaaatgccgcaaaaaagggaataagggcgacacggaaatgttgaatactcatactcttcctttttcaatattattgaagcatttatcagggttattgtctcatgagcggatacatatttgaatgtatttagaaaaataaacaaataggggttccgcgcacatttccccgaaaagtgccacctaaattgtaagcgttaatattttgttaaaattcgcgttaaatttttgttaaatcagctcattttttaaccaataggccgaaatcggcaaaatcccttataaatcaaaagaatagaccgagatagggttgagtggccgctacagggcgctcccattcgccattcaggctgcgcaactgttgggaagggcgtttcggtgcgggcctcttcgctattacgccagctggcgaaagggggatgtgctgcaaggcgattaagttgggtaacgccagggttttcccagtcacgacgttgtaaaacgacggccagtgagcgcgacgtaatacgactcactatagggcgaattggcggaaggccgtcaaggccgcatgaattcgctaccgggaagttcctattccgaagttcctattctatcagaagtataggaacttcaggtacgccaccatgctccttgaacatttattaataatcttgtggatgcagctgacatgggtcagtggtcaacagctgaatcagagtcctcaatctatgtttatccaggaaggagaagatgtctccatgaactgcacttcttcaagcatatttaacacctggctatggtacaagcaggaacctggggaaggtcctgtcctcttgatagccttatataaggctggtgaattgacctcaaatggaaggctgactgctcagtttggtataaccagaaaggacagcttcctgaatatctcagcatccatacctagtgatgtaggcatctacttctgcgctggacccangaaancctccnacgacaaggtgatatttgggccagggacaagcttatcagtcattccaaatatccagaaccctgaccctgccgtgtaccagctgagagactctaaatccagtgacaagtctgtctgcctattcaccgattttgattctcaaacaaatgtgtcacaaagtaaggattctgatgtgtatatcacagacaaaactgtgctagacatgaggtctatggacttcaagagcaacagtgctgtggcctggagcaacaaatctgactttgcatgtgcaaacgccttcaacaacagcattattccagaggacaccttcttccccagcccagaaagttcctgtgatgtcaagctggtcgagaaaagctttgaaacagatacgaacctaaactttcaaaacctgtcagtgattgggttccgaatcctcctcctgaaagtggccgggtttaatctgctcatgacgctgcggctgtggtccagctgactag

SEQ ID NO: 13 - DNA, 4542 bp, Artificial Sequence
  CMVpro-Flp-sv40pA-V2 vector V4.I.8
ctaaattgtaagcgttaatattttgttaaaattcgcgttaaatttttgttaaatcagctcattttttaaccaataggccgaaatcggcaaaatcccttataaatcaaaagaatagaccgagatagggttgagtggccgctacagggcgctcccattcgccattcaggctgcgcaactgttgggaagggcgtttcggtgcgggcctcttcgctattacgccagctggcgaaagggggatgtgctgcaaggcgattaagttgggtaacgccagggttttcccagtcacgacgttgtaaaacgacggccagtgagcgcgacgtaatacgactcactatagggcgaattggcggaaggccgtcaaggccgcatgaattcgctaccggtatagtaatcaattacggggtcattagttcatagcccatatatggagttccgcgttacataacttacggtaaatggcccgcctggctgaccgcccaacgacccccgcccattgacgtcaataatgacgtatgttcccatagtaacgccaatagggactttccattgacgtcaatgggtggagtatttacggtaaactgcccacttggcagtacatcaagtgtatcatatgccaagtacgccccctattgacgtcaatgacggtaaatggcccgcctggcattatgcccagtacatgaccttatgggactttcctacttggcagtacatctacgtattagtcatcgctattaccatggtgatgcggttttggcagtacatcaatgggcgtggatagcggtttgactcacggggatttccaagtctccaccccattgacgtcaatgggagtttgttttggcaccaaaatcaacgggactttccaaaatgtcgtaacaactccgccccattgacgcaaatgggcggtaggcgtgtacggtgggaggtctatataagcagagctggtttagtgaaccgtcagatcaggtaccatggcccccaagaaaaagcggaaagtgggcatccacggcgtgccagctgcaggcggctctatgagccagttcgacatcctgtgcaagaccccacctaaggtgctcgtgcggcagttcgtggaaagattcgagaggcctagcggcgagaagatcgcctcttgtgctgccgagctgacctacctgtgctggatgatcacccacaacggcaccgccatcaagcgggccaccttcatgagctacaataccatcatcagcaacagcctgagcttcgacatcgtgaacaagagcctgcagttcaagtacaagacccagaaggccaccatcctggaagccagcctgaagaaactgatccccgcctgggagtttaccatcatcccatacaatggccagaaacatcagagcgacattaccgatatcgtgtccagcctccagctgcagttcgagagtagcgaagaagccgacaagggcaacagccacagcaagaagatgctgaaggccctgctgagcgagggcgagagcatctgggagatcacagagaagatcctgaacagcttcgagtacaccagccggttcaccaagaccaagaccctgtaccagttcctgttcctggccacctttatcaactgcggccggttctccgacatcaagaacgtggaccccaagagcttcaagctggtgcagaacaagtacctgggcgtgatcattcagtgcctcgtgaccgagacaaagaccagcgtgtcccggcacatctactttttcagcgccagaggccggatcgaccccctggtgtacctggacgagttcctgagaaacagcgagcccgtgctgaagagagtgaaccggaccggcaacagcagctccaacaagcaggaataccagctgctgaaggacaacctcgtgcggtcctacaacaaggccctgaagaaaaacgccccctaccccatcttcgccattaagaacggccccaagtcccacatcggccggcacctgatgaccagctttctgagcatgaagggcctgacagagctgaccaacgtcgtgggcaattggagcgacaagagggcctctgccgtggccagaaccacctacacccaccagatcacagccatccccgaccactacttcgccctggtgtctcggtactacgcctacgaccccatcagcaaagagatgatcgccctgaaggacgagacaaaccccatcgaggaatggcagcacatcgagcagctgaagggcagcgccgagggcagcatcagataccctgcctggaacggcatcatctcccaggaagtgctggactacctgagcagctacatcaaccggcggatctgatctagacctgatcataatcaagccatatcacatctgtagaggtttacttgctttaaaaaacctccacacctccccctgaacctgaaacataaaatgaatgcaattgttgttgttaacttgtttattgcagcttataatggttacaaataaagcaatagcatcacaaatttcacaaataaagcatttttttcactgcattctagttgtggtttgtccaaactcatcaatgtatcttatcatgtctggatctgcggatccaatctcgagctgggcctcatgggccttccgctcactgcccgctttccagtcgggaaacctgtcgtgccagctgcattaacatggtcatagctgtttccttgcgtattgggcgctctccgcttcctcgctcactgactcgctgcgctcggtcgttcgggtaaagcctggggtgcctaatgagcaaaaggccagcaaaaggccaggaaccgtaaaaaggccgcgttgctggcgtttttccataggctccgcccccctgacgagcatcacaaaaatcgacgctcaagtcagaggtggcgaaacccgacaggactataaagataccaggcgtttccccctggaagctccctcgtgcgctctcctgttccgaccctgccgcttaccggatacctgtccgcctttctcccttcgggaagcgtggcgctttctcatagctcacgctgtaggtatctcagttcggtgtaggtcgttcgctccaagctgggctgtgtgcacgaaccccccgttcagcccgaccgctgcgccttatccggtaactatcgtcttgagtccaacccggtaagacacgacttatcgccactggcagcagccactggtaacaggattagcagagcgaggtatgtaggcggtgctacagagttcttgaagtggtggcctaactacggctacactagaagaacagtatttggtatctgcgctctgctgaagccagttaccttcggaaaaagagttggtagctcttgatccggcaaacaaaccaccgctggtagcggtggtttttttgtttgcaagcagcagattacgcgcagaaaaaaaggatctcaagaagatcctttgatcttttctacggggtctgacgctcagtggaacgaaaactcacgttaagggattttggtcatgagattatcaaaaaggatcttcacctagatccttttaaattaaaaatgaagttttaaatcaatctaaagtatatatgagtaaacttggtctgacagttaccaatgcttaatcagtgaggcacctatctcagcgatctgtctatttcgttcatccatagttgcctgactccccgtcgtgtagataactacgatacgggagggcttaccatctggccccagtgctgcaatgataccgcgagaaccacgctcaccggctccagatttatcagcaataaaccagccagccggaagggccgagcgcagaagtggtcctgcaactttatccgcctccatccagtctattaattgttgccgggaagctagagtaagtagttcgccagttaatagtttgcgcaacgttgttgccattgctacaggcatcgtggtgtcacgctcgtcgtttggtatggcttcattcagctccggttcccaacgatcaaggcgagttacatgatcccccatgttgtgcaaaaaagcggttagctccttcggtcctccgatcgttgtcagaagtaagttggccgcagtgttatcactcatggttatggcagcactgcataattctcttactgtcatgccatccgtaagatgcttttctgtgactggtgagtactcaaccaagtcattctgagaatagtgtatgcggcgaccgagttgctcttgcccggcgtcaatacgggataataccgcgccacatagcagaactttaaaagtgctcatcattggaaaacgttcttcggggcgaaaactctcaaggatcttaccgctgttgagatccagttcgatgtaacccactcgtgcacccaactgatcttcagcatcttttactttcaccagcgtttctgggtgagcaaaaacaggaaggcaaaatgccgcaaaaaagggaataagggcgacacggaaatgttgaatactcatactcttcctttttcaatattattgaagcatttatcagggttattgtctcatgagcggatacatatttgaatgtatttagaaaaataaacaaataggggttccgcgcacatttccccgaaaagtgccac

SEQ ID NO: 14 - DNA, 42 bp, Artificial Sequence
  CDR3 sequence of a JG9-TRA 64 variant VP.7751.RC1_A1
tgcgctggacccaagaaaacctccaacgacaaggtgatattt

SEQ ID NO: 15 - DNA, 42 bp, Artificial Sequence
  CDR3 sequence of a JG9-TRA 64 variant VP.7751.RC1_A2
tgcgctggacccaagaaaacctcccacgacaaggtgatattt

SEQ ID NO: 16 - DNA, 42 bp, Artificial Sequence
  CDR3 sequence of a JG9-TRA 64 variant VP.7751.RC1_A3
tgcgctggacccaagaaaacctccgacgacaaggtgatattt

SEQ ID NO: 17 - DNA, 42 bp, Artificial Sequence
  CDR3 sequence of a JG9-TRA 64 variant VP.7751.RC1_A4
tgcgctggacccaagaaaacctcctacgacaaggtgatattt

SEQ ID NO: 18 - DNA, 42 bp, Artificial Sequence
  CDR3 sequence of a JG9-TRA 64 variant VP.7751.RC1_A5
tgcgctggacccaagaaaccctccaacgacaaggtgatattt

SEQ ID NO: 19 - DNA, 42 bp, Artificial Sequence
  CDR3 sequence of a JG9-TRA 64 variant VP.7751.RC1_A6
tgcgctggacccaagaaaccctcccacgacaaggtgatattt

SEQ ID NO: 20 - DNA, 42 bp, Artificial Sequence
  CDR3 sequence of a JG9-TRA 64 variant VP.7751.RC1_A7
tgcgctggacccaagaaaccctccgacgacaaggtgatattt

SEQ ID NO: 21 - DNA, 42 bp, Artificial Sequence
  CDR3 sequence of a JG9-TRA 64 variant VP.7751.RC1_A8
tgcgctggacccaagaaaccctcctacgacaaggtgatattt

SEQ ID NO: 22 - DNA, 42 bp, Artificial Sequence
  CDR3 sequence of a JG9-TRA 64 variant VP.7751.RC1_B1
tgcgctggacccaagaaagcctccaacgacaaggtgatattt

SEQ ID NO: 23 - DNA, 42 bp, Artificial Sequence
  CDR3 sequence of a JG9-TRA 64 variant VP.7751.RC1_B2
tgcgctggacccaagaaagcctcccacgacaaggtgatattt

SEQ ID NO: 24 - DNA, 42 bp, Artificial Sequence
  CDR3 sequence of a JG9-TRA 64 variant VP.7751.RC1_B3
tgcgctggacccaagaaagcctccgacgacaaggtgatattt

SEQ ID NO: 25 - DNA, 42 bp, Artificial Sequence
  CDR3 sequence of a JG9-TRA 64 variant VP.7751.RC1_B4
tgcgctggacccaagaaagcctcctacgacaaggtgatattt

SEQ ID NO: 26 - DNA, 42 bp, Artificial Sequence
  CDR3 sequence of a JG9-TRA 64 variant VP.7751.RC1_B5
tgcgctggacccaagaaatcctccaacgacaaggtgatattt

SEQ ID NO: 27 - DNA, 42 bp, Artificial Sequence
  CDR3 sequence of a JG9-TRA 64 variant VP.7751.RC1_B6
tgcgctggacccaagaaatcctcccacgacaaggtgatattt

SEQ ID NO: 28 - DNA, 42 bp, Artificial Sequence
  CDR3 sequence of a JG9-TRA 64 variant VP.7751.RC1_B7
tgcgctggacccaagaaatcctccgacgacaaggtgatattt

SEQ ID NO: 29 - DNA, 42 bp, Artificial Sequence
  CDR3 sequence of a JG9-TRA 64 variant VP.7751.RC1_B8
tgcgctggacccaagaaatcctcctacgacaaggtgatattt

SEQ ID NO: 30 - DNA, 42 bp, Artificial Sequence
  CDR3 sequence of a JG9-TRA 64 variant VP.7751.RC1_C1
tgcgctggacccacgaaaacctccaacgacaaggtgatattt

SEQ ID NO: 31 - DNA, 42 bp, Artificial Sequence
  CDR3 sequence of a JG9-TRA 64 variant VP.7751.RC1_C2
tgcgctggacccacgaaaacctcccacgacaaggtgatattt

SEQ ID NO: 32 - DNA, 42 bp, Artificial Sequence
  CDR3 sequence of a JG9-TRA 64 variant VP.7751.RC1_C3
tgcgctggacccacgaaaacctccgacgacaaggtgatattt

SEQ ID NO: 33 - DNA, 42 bp, Artificial Sequence
  CDR3 sequence of a JG9-TRA 64 variant VP.7751.RC1_C4
tgcgctggacccacgaaaacctcctacgacaaggtgatattt

SEQ ID NO: 34 - DNA, 42 bp, Artificial Sequence
  CDR3 sequence of a JG9-TRA 64 variant VP.7751.RC1_C5
tgcgctggacccacgaaaccctccaacgacaaggtgatattt

SEQ ID NO: 35 - DNA, 42 bp, Artificial Sequence
  CDR3 sequence of a JG9-TRA 64 variant VP.7751.RC1_C6
tgcgctggacccacgaaaccctcccacgacaaggtgatattt

SEQ ID NO: 36 - DNA, 42 bp, Artificial Sequence
  CDR3 sequence of a JG9-TRA 64 variant VP.7751.RC1_C7
tgcgctggacccacgaaaccctcctacgacaaggtgatattt

SEQ ID NO: 37 - DNA, 42 bp, Artificial Sequence
  CDR3 sequence of a JG9-TRA 64 variant VP.7751.RC1_D1
tgcgctggacccacgaaagcctccaacgacaaggtgatattt

SEQ ID NO: 38 - DNA, 42 bp, Artificial Sequence
  CDR3 sequence of a JG9-TRA 64 variant VP.7751.RC1_D2
tgcgctggacccacgaaagcctcccacgacaaggtgatattt

SEQ ID NO: 39 - DNA, 42 bp, Artificial Sequence
  CDR3 sequence of a JG9-TRA 64 variant VP.7751.RC1_D3
tgcgctggacccacgaaagcctccgacgacaaggtgatattt

SEQ ID NO: 40 - DNA, 42 bp, Artificial Sequence
  CDR3 sequence of a JG9-TRA 64 variant VP.7751.RC1_D4
tgcgctggacccacgaaagcctcctacgacaaggtgatattt

SEQ ID NO: 41 - DNA, 42 bp, Artificial Sequence
  CDR3 sequence of a JG9-TRA 64 variant VP.7751.RC1_D5
tgcgctggacccacgaaatcctccaacgacaaggtgatattt

SEQ ID NO: 42 - DNA, 42 bp, Artificial Sequence
  CDR3 sequence of a JG9-TRA 64 variant VP.7751.RC1_D6
tgcgctggacccacgaaatcctcccacgacaaggtgatattt

SEQ ID NO: 43 - DNA, 42 bp, Artificial Sequence
  CDR3 sequence of a JG9-TRA 64 variant VP.7751.RC1_D7
tgcgctggacccacgaaatcctccgacgacaaggtgatattt

SEQ ID NO: 44 - DNA, 42 bp, Artificial Sequence
  CDR3 sequence of a JG9-TRA 64 variant VP.7751.RC1_D8
tgcgctggacccacgaaatcctcctacgacaaggtgatattt

SEQ ID NO: 45 - DNA, 42 bp, Artificial Sequence
  CDR3 sequence of a JG9-TRA 64 variant VP.7751.RC1_E1
tgcgctggacccaggaaaacctccaacgacaaggtgatattt

SEQ ID NO: 46 - DNA, 42 bp, Artificial Sequence
  CDR3 sequence of a JG9-TRA 64 variant VP.7751.RC1_E2
tgcgctggacccaggaaaacctcccacgacaaggtgatattt

SEQ ID NO: 47 - DNA, 42 bp, Artificial Sequence
  CDR3 sequence of a JG9-TRA 64 variant VP.7751.RC1_E3
tgcgctggacccaggaaaacctccgacgacaaggtgatattt

SEQ ID NO: 48 - DNA, 42 bp, Artificial Sequence
  CDR3 sequence of a JG9-TRA 64 variant VP.7751.RC1_E4
tgcgctggacccaggaaaacctcctacgacaaggtgatattt

SEQ ID NO: 49 - DNA, 42 bp, Artificial Sequence
  CDR3 sequence of a JG9-TRA 64 variant VP.7751.RC1_E5
tgcgctggacccaggaaaccctccaacgacaaggtgatattt

SEQ ID NO: 50 - DNA, 42 bp, Artificial Sequence
  CDR3 sequence of a JG9-TRA 64 variant VP.7751.RC1_E6
tgcgctggacccaggaaaccctcccacgacaaggtgatattt

SEQ ID NO: 51 - DNA, 42 bp, Artificial Sequence
  CDR3 sequence of a JG9-TRA 64 variant VP.7751.RC1_E7
tgcgctggacccaggaaaccctccgacgacaaggtgatattt

SEQ ID NO: 52 - protein, 42 aa, Artificial Sequence
  CDR3 sequence of a JG9-TRA 64 variant VP.7751.RC1_E8
TGCGCTGGACCCAGGAAACCCTCCTACGACAAGGTGATATTT

SEQ ID NO: 53 - DNA, 42 bp, Artificial Sequence
  CDR3 sequence of a JG9-TRA 64 variant VP.7751.RC1_F1
tgcgctggacccaggaaagcctccaacgacaaggtgatattt

SEQ ID NO: 54 - DNA, 42 bp, Artificial Sequence
  CDR3 sequence of a JG9-TRA 64 variant VP.7751.RC1_F2
tgcgctggacccaggaaagcctcccacgacaaggtgatattt

SEQ ID NO: 55 - DNA, 42 bp, Artificial Sequence
  CDR3 sequence of a JG9-TRA 64 variant VP.7751.RC1_F3
tgcgctggacccaggaaagcctccgacgacaaggtgatattt

SEQ ID NO: 56 - DNA, 42 bp, Artificial Sequence
  CDR3 sequence of a JG9-TRA 64 variant VP.7751.RC1_F4
tgcgctggacccaggaaagcctcctacgacaaggtgatattt

SEQ ID NO: 57 - DNA, 42 bp, Artificial Sequence
  CDR3 sequence of a JG9-TRA 64 variant VP.7751.RC1_F5
tgcgctggacccaggaaatcctccaacgacaaggtgatattt

SEQ ID NO: 58 - DNA, 42 bp, Artificial Sequence
  CDR3 sequence of a JG9-TRA 64 variant VP.7751.RC1_F6
tgcgctggacccaggaaatcctcccacgacaaggtgatattt

SEQ ID NO: 59 - DNA, 42 bp, Artificial Sequence
  CDR3 sequence of a JG9-TRA 64 variant VP.7751.RC1_F7
tgcgctggacccaggaaatcctccgacgacaaggtgatattt

SEQ ID NO: 60 - DNA, 42 bp, Artificial Sequence
  CDR3 sequence of a JG9-TRA 64 variant VP.7751.RC1_F8
tgcgctggacccaggaaatcctcctacgacaaggtgatattt

SEQ ID NO: 61 - DNA, 42 bp, Artificial Sequence
  CDR3 sequence of a JG9-TRA 64 variant VP.7751.RC1_G1
tgcgctggacccatgaaaacctccaacgacaaggtgatattt

SEQ ID NO: 62 - DNA, 42 bp, Artificial Sequence
  CDR3 sequence of a JG9-TRA 64 variant VP.7751.RC1_G2
tgcgctggacccatgaaaacctcccacgacaaggtgatattt

SEQ ID NO: 63 - DNA, 42 bp, Artificial Sequence
  CDR3 sequence of a JG9-TRA 64 variant VP.7751.RC1_G3
tgcgctggacccatgaaaacctccgacgacaaggtgatattt

SEQ ID NO: 64 - DNA, 42 bp, Artificial Sequence
  CDR3 sequence of a JG9-TRA 64 variant VP.7751.RC1_G4
tgcgctggacccatgaaaacctcctacgacaaggtgatattt

SEQ ID NO: 65 - DNA, 42 bp, Artificial Sequence
  CDR3 sequence of a JG9-TRA 64 variant VP.7751.RC1_G5
tgcgctggacccatgaaaccctccaacgacaaggtgatattt

SEQ ID NO: 66 - DNA, 42 bp, Artificial Sequence
  CDR3 sequence of a JG9-TRA 64 variant VP.7751.RC1_G6
tgcgctggacccatgaaaccctcccacgacaaggtgatattt

SEQ ID NO: 67 - DNA, 42 bp, Artificial Sequence
  CDR3 sequence of a JG9-TRA 64 variant VP.7751.RC1_G7
tgcgctggacccatgaaaccctccgacgacaaggtgatattt

SEQ ID NO: 68 - DNA, 42 bp, Artificial Sequence
  CDR3 sequence of a JG9-TRA 64 variant VP.7751.RC1_G8
tgcgctggacccatgaaaccctcctacgacaaggtgatattt

SEQ ID NO: 69 - DNA, 42 bp, Artificial Sequence
  CDR3 sequence of a JG9-TRA 64 variant VP.7751.RC1_H1
tgcgctggacccatgaaagcctccaacgacaaggtgatattt

SEQ ID NO: 70 - DNA, 42 bp, Artificial Sequence
  CDR3 sequence of a JG9-TRA 64 variant VP.7751.RC1_H2
tgcgctggacccatgaaagcctcccacgacaaggtgatattt

SEQ ID NO: 71 - DNA, 42 bp, Artificial Sequence
  CDR3 sequence of a JG9-TRA 64 variant VP.7751.RC1_H3
tgcgctggacccatgaaagcctccgacgacaaggtgatattt

SEQ ID NO: 72 - DNA, 42 bp, Artificial Sequence
  CDR3 sequence of a JG9-TRA 64 variant VP.7751.RC1_H4
tgcgctggacccatgaaagcctcctacgacaaggtgatattt

SEQ ID NO: 73 - DNA, 42 bp, Artificial Sequence
  CDR3 sequence of a JG9-TRA 64 variant VP.7751.RC1_H5
tgcgctggacccatgaaatcctccaacgacaaggtgatattt

SEQ ID NO: 74 - DNA, 42 bp, Artificial Sequence
  CDR3 sequence of a JG9-TRA 64 variant VP.7751.RC1_H6
tgcgctggacccatgaaatcctcccacgacaaggtgatattt

SEQ ID NO: 75 - DNA, 42 bp, Artificial Sequence
  CDR3 sequence of a JG9-TRA 64 variant VP.7751.RC1_H7
tgcgctggacccatgaaatcctccgacgacaaggtgatattt

SEQ ID NO: 76 - DNA, 42 bp, Artificial Sequence
  CDR3 sequence of a JG9-TRA 64 variant VP.7751.RC1_H8
tgcgctggacccatgaaatcctcctacgacaaggtgatattt

SEQ ID NO: 77 - DNA, 3602 bp, Artificial Sequence
  pMA_F14_HLA-A*02:01-6xHis_F15 vector V4.H.5
ctaaattgtaagcgttaatattttgttaaaattcgcgttaaatttttgttaaatcagctcattttttaaccaataggccgaaatcggcaaaatcccttataaatcaaaagaatagaccgagatagggttgagtggccgctacagggcgctcccattcgccattcaggctgcgcaactgttgggaagggcgtttcggtgcgggcctcttcgctattacgccagctggcgaaagggggatgtgctgcaaggcgattaagttgggtaacgccagggttttcccagtcacgacgttgtaaaacgacggccagtgagcgcgacgtaatacgactcactatagggcgaattggcggaaggccgtcaaggccgcatgaattcgctaccgggaagttcctattccgaagttcctattctatcagaagtataggaacttcaggtaccatggccgtcatggcgccccgaaccctcgtcctgctactctcgggggctctggccctgacccagacctgggcgggctctcactccatgaggtatttcttcacatccgtgtctcggccaggacgcggagagccacgcttcatcgcagtgggctacgtggacgacacgcagttcgtgcggttcgacagcgacgccgcgagccagaggatggagccgcgggcgccgtggatagagcaggagggtccggagtattgggacggggagacacggaaagtgaaggcccactcacagactcaccgagtggacctggggaccctgcgcggctactacaaccagagcgaggccggttctcacaccgtccagaggatgtatggctgcgacgtggggtcggactggcgcttcctccgcggataccaccagtacgcctacgacggcaaggattacatcgccctgaaagaggacctgcgctcttggaccgcggcggacatggcagctcagaccaccaagcacaagtgggaggcggcccatgtggcggagcagttgagagcctacctggagggcacgtgcgtggagtggctccgcagatacctggagaacgggaaggagacgctgcagcgcacggacgcccccaaaacgcatatgactcaccacgctgtctctgaccatgaagccaccctgaggtgctgggccctgagcttctaccctgcggagatcacactgacctggcagcgggatggggaggaccagacccaggacacggagctcgtggagaccaggcctgcaggggatggaaccttccagaagtgggcggctgtggtggtgccttctggacaggagcagagatacacctgccatgtgcagcatgagggtttgcccaagcccctcaccctgagatgggagccgtcttcccagcccaccatccccatcgtgggcatcattgctggcctggttctctttggagctgtgatcactggagctgtggtcgctgctgtgatgtggaggaggaagagctcagatagaaaaggagggagctactctcaggctgcaagcagtgacagtgcccagggctctgatgtgtctctcacagcttgtaaagtgcccgggcatcatcaccatcaccactgactatagtcgtctagacgaagttcctattccgaagttcctattcttataggagtataggaacttcctcgagctgggcctcatgggccttccgctcactgcccgctttccagtcgggaaacctgtcgtgccagctgcattaacatggtcatagctgtttccttgcgtattgggcgctctccgcttcctcgctcactgactcgctgcgctcggtcgttcgggtaaagcctggggtgcctaatgagcaaaaggccagcaaaaggccaggaaccgtaaaaaggccgcgttgctggcgtttttccataggctccgcccccctgacgagcatcacaaaaatcgacgctcaagtcagaggtggcgaaacccgacaggactataaagataccaggcgtttccccctggaagctccctcgtgcgctctcctgttccgaccctgccgcttaccggatacctgtccgcctttctcccttcgggaagcgtggcgctttctcatagctcacgctgtaggtatctcagttcggtgtaggtcgttcgctccaagctgggctgtgtgcacgaaccccccgttcagcccgaccgctgcgccttatccggtaactatcgtcttgagtccaacccggtaagacacgacttatcgccactggcagcagccactggtaacaggattagcagagcgaggtatgtaggcggtgctacagagttcttgaagtggtggcctaactacggctacactagaagaacagtatttggtatctgcgctctgctgaagccagttaccttcggaaaaagagttggtagctcttgatccggcaaacaaaccaccgctggtagcggtggtttttttgtttgcaagcagcagattacgcgcagaaaaaaaggatctcaagaagatcctttgatcttttctacggggtctgacgctcagtggaacgaaaactcacgttaagggattttggtcatgagattatcaaaaaggatcttcacctagatccttttaaattaaaaatgaagttttaaatcaatctaaagtatatatgagtaaacttggtctgacagttaccaatgcttaatcagtgaggcacctatctcagcgatctgtctatttcgttcatccatagttgcctgactccccgtcgtgtagataactacgatacgggagggcttaccatctggccccagtgctgcaatgataccgcgagaaccacgctcaccggctccagatttatcagcaataaaccagccagccggaagggccgagcgcagaagtggtcctgcaactttatccgcctccatccagtctattaattgttgccgggaagctagagtaagtagttcgccagttaatagtttgcgcaacgttgttgccattgctacaggcatcgtggtgtcacgctcgtcgtttggtatggcttcattcagctccggttcccaacgatcaaggcgagttacatgatcccccatgttgtgcaaaaaagcggttagctccttcggtcctccgatcgttgtcagaagtaagttggccgcagtgttatcactcatggttatggcagcactgcataattctcttactgtcatgccatccgtaagatgcttttctgtgactggtgagtactcaaccaagtcattctgagaatagtgtatgcggcgaccgagttgctcttgcccggcgtcaatacgggataataccgcgccacatagcagaactttaaaagtgctcatcattggaaaacgttcttcggggcgaaaactctcaaggatcttaccgctgttgagatccagttcgatgtaacccactcgtgcacccaactgatcttcagcatcttttactttcaccagcgtttctgggtgagcaaaaacaggaaggcaaaatgccgcaaaaaagggaataagggcgacacggaaatgttgaatactcatactcttcctttttcaatattattgaagcatttatcagggttattgtctcatgagcggatacatatttgaatgtatttagaaaaataaacaaataggggttccgcgcacatttccccgaaaagtgccac

SEQ ID NO: 78 - DNA, 3602 bp, Artificial Sequence
  pMA_F14_HLA-A*24:02-6xHis_F15 vector V4.H.6
ctaaattgtaagcgttaatattttgttaaaattcgcgttaaatttttgttaaatcagctcattttttaaccaataggccgaaatcggcaaaatcccttataaatcaaaagaatagaccgagatagggttgagtggccgctacagggcgctcccattcgccattcaggctgcgcaactgttgggaagggcgtttcggtgcgggcctcttcgctattacgccagctggcgaaagggggatgtgctgcaaggcgattaagttgggtaacgccagggttttcccagtcacgacgttgtaaaacgacggccagtgagcgcgacgtaatacgactcactatagggcgaattggcggaaggccgtcaaggccgcatgaattcgctaccgggaagttcctattccgaagttcctattctatcagaagtataggaacttcaggtaccatggccgtcatggcgccccgaaccctcgtcctgctactctcgggggccctggccctgacccagacctgggcaggctcccactccatgaggtatttctccacatccgtgtctcggccaggacgcggagagccacgcttcatcgccgtgggctacgtggacgacacgcagttcgtgcggttcgacagcgacgccgcgagccagaggatggagccgcgggcgccgtggatagagcaggaggggccggagtattgggacgaggagacagggaaagtgaaggcccactcacagactgaccgagagaacctgcggatcgcgctccgctactacaaccagagcgaggccggttctcacaccctccagatgatgtttggctgcgacgtggggtcggacgggcgcttcctccgcggataccaccagtacgcctacgacggcaaggattacatcgccctgaaagaggacctgcgctcttggaccgcggcggacatggcggctcagatcaccaagcgcaagtgggaggcggcccatgtggcggagcagcagagagcctacctggagggcacgtgcgtggacgggctccgcagatacctggagaacgggaaggagacgctgcagcgcacggacccccccaagacacatatgacccaccaccccatctctgaccatgaggccactctgagatgctgggccctgggcttctaccctgcggagatcacactgacctggcagcgggatggggaggaccagacccaggacacggagcttgtggagaccaggcctgcaggggatggaaccttccagaagtgggcagctgtggtggttccttctggagaggagcagagatacacctgccatgtgcagcatgagggtctgcccaagcccctcaccctgagatgggagccatcttcccagcccaccgtccccatcgtgggcatcattgctggcctggttctccttggagctgtgatcactggagctgtggtcgctgctgtgatgtggaggaggaacagctcagatagaaaaggagggagctactctcaggctgcaagcagtgacagtgcccagggctctgatgtgtctctcacagcttgtaaagtgcccgggcatcatcaccatcaccactgactatagtcgtctagacgaagttcctattccgaagttcctattcttataggagtataggaacttcctcgagctgggcctcatgggccttccgctcactgcccgctttccagtcgggaaacctgtcgtgccagctgcattaacatggtcatagctgtttccttgcgtattgggcgctctccgcttcctcgctcactgactcgctgcgctcggtcgttcgggtaaagcctggggtgcctaatgagcaaaaggccagcaaaaggccaggaaccgtaaaaaggccgcgttgctggcgtttttccataggctccgcccccctgacgagcatcacaaaaatcgacgctcaagtcagaggtggcgaaacccgacaggactataaagataccaggcgtttccccctggaagctccctcgtgcgctctcctgttccgaccctgccgcttaccggatacctgtccgcctttctcccttcgggaagcgtggcgctttctcatagctcacgctgtaggtatctcagttcggtgtaggtcgttcgctccaagctgggctgtgtgcacgaaccccccgttcagcccgaccgctgcgccttatccggtaactatcgtcttgagtccaacccggtaagacacgacttatcgccactggcagcagccactggtaacaggattagcagagcgaggtatgtaggcggtgctacagagttcttgaagtggtggcctaactacggctacactagaagaacagtatttggtatctgcgctctgctgaagccagttaccttcggaaaaagagttggtagctcttgatccggcaaacaaaccaccgctggtagcggtggtttttttgtttgcaagcagcagattacgcgcagaaaaaaaggatctcaagaagatcctttgatcttttctacggggtctgacgctcagtggaacgaaaactcacgttaagggattttggtcatgagattatcaaaaaggatcttcacctagatccttttaaattaaaaatgaagttttaaatcaatctaaagtatatatgagtaaacttggtctgacagttaccaatgcttaatcagtgaggcacctatctcagcgatctgtctatttcgttcatccatagttgcctgactccccgtcgtgtagataactacgatacgggagggcttaccatctggccccagtgctgcaatgataccgcgagaaccacgctcaccggctccagatttatcagcaataaaccagccagccggaagggccgagcgcagaagtggtcctgcaactttatccgcctccatccagtctattaattgttgccgggaagctagagtaagtagttcgccagttaatagtttgcgcaacgttgttgccattgctacaggcatcgtggtgtcacgctcgtcgtttggtatggcttcattcagctccggttcccaacgatcaaggcgagttacatgatcccccatgttgtgcaaaaaagcggttagctccttcggtcctccgatcgttgtcagaagtaagttggccgcagtgttatcactcatggttatggcagcactgcataattctcttactgtcatgccatccgtaagatgcttttctgtgactggtgagtactcaaccaagtcattctgagaatagtgtatgcggcgaccgagttgctcttgcccggcgtcaatacgggataataccgcgccacatagcagaactttaaaagtgctcatcattggaaaacgttcttcggggcgaaaactctcaaggatcttaccgctgttgagatccagttcgatgtaacccactcgtgcacccaactgatcttcagcatcttttactttcaccagcgtttctgggtgagcaaaaacaggaaggcaaaatgccgcaaaaaagggaataagggcgacacggaaatgttgaatactcatactcttcctttttcaatattattgaagcatttatcagggttattgtctcatgagcggatacatatttgaatgtatttagaaaaataaacaaataggggttccgcgcacatttccccgaaaagtgccac

SEQ ID NO: 79 - DNA, 3593 bp, Artificial Sequence
  pMA_F14_HLA-B*07:02-6xHis_F15 vector V4.H.7
ctaaattgtaagcgttaatattttgttaaaattcgcgttaaatttttgttaaatcagctcattttttaaccaataggccgaaatcggcaaaatcccttataaatcaaaagaatagaccgagatagggttgagtggccgctacagggcgctcccattcgccattcaggctgcgcaactgttgggaagggcgtttcggtgcgggcctcttcgctattacgccagctggcgaaagggggatgtgctgcaaggcgattaagttgggtaacgccagggttttcccagtcacgacgttgtaaaacgacggccagtgagcgcgacgtaatacgactcactatagggcgaattggcggaaggccgtcaaggccgcatgaattcgctaccgggaagttcctattccgaagttcctattctatcagaagtataggaacttcaggtaccatgctggtcatggcgccccgaaccgtcctcctgctgctctcggcggccctggccctgaccgagacctgggccggctcccactccatgaggtatttctacacctccgtgtctcggccaggacgcggagagccacgcttcatctcagtgggctacgtggacgacacccagttcgtgaggttcgacagcgacgccgcgagtccgagagaggagccgcgggcgccgtggatagagcaggaggggccggagtattgggaccggaacacacagatctacaaggcccaggcacagactgaccgagagagcctgcggaacctgcgcggctactacaaccagagcgaggccgggtctcacaccctccagagcatgtacggctgcgacgtggggccggacgggcgcctcctccgcgggcatgaccagtacgcctacgacggcaaggattacatcgccctgaacgaggacctgcgctcctggaccgccgcggacacggcggctcagatcacccagcgcaagtgggaggcggcccgtgaggcggagcagcggagagcctacctggagggcgagtgcgtggagtggctccgcagatacctggagaacgggaaggacaaacttgagcgcgcagaccctccaaagacacacgtgacccaccaccccatctctgaccatgaggccaccctgaggtgctgggccctgggtttctaccctgcggagatcacactgacctggcagcgggatggcgaggaccaaactcaggacactgagcttgtggagaccagaccagcaggagatagaaccttccagaagtgggcagctgtggtggtgccttctggagaagagcagagatacacatgccatgtacagcatgaggggctgccgaagcccctcaccctgagatgggagccgtcttcccagtccaccgtccccatcgtgggcattgttgctggcctggctgtcctagcagttgtggtcatcggagctgtggtcgctgctgtgatgtgtaggaggaagagttcaggtggaaaaggagggagctactctcaggctgcgtgcagcgacagtgcccagggctctgatgtgtctctcacagctcccgggcatcatcaccatcaccactgactatagtcgtctagacgaagttcctattccgaagttcctattcttataggagtataggaacttcctcgagctgggcctcatgggccttccgctcactgcccgctttccagtcgggaaacctgtcgtgccagctgcattaacatggtcatagctgtttccttgcgtattgggcgctctccgcttcctcgctcactgactcgctgcgctcggtcgttcgggtaaagcctggggtgcctaatgagcaaaaggccagcaaaaggccaggaaccgtaaaaaggccgcgttgctggcgtttttccataggctccgcccccctgacgagcatcacaaaaatcgacgctcaagtcagaggtggcgaaacccgacaggactataaagataccaggcgtttccccctggaagctccctcgtgcgctctcctgttccgaccctgccgcttaccggatacctgtccgcctttctcccttcgggaagcgtggcgctttctcatagctcacgctgtaggtatctcagttcggtgtaggtcgttcgctccaagctgggctgtgtgcacgaaccccccgttcagcccgaccgctgcgccttatccggtaactatcgtcttgagtccaacccggtaagacacgacttatcgccactggcagcagccactggtaacaggattagcagagcgaggtatgtaggcggtgctacagagttcttgaagtggtggcctaactacggctacactagaagaacagtatttggtatctgcgctctgctgaagccagttaccttcggaaaaagagttggtagctcttgatccggcaaacaaaccaccgctggtagcggtggtttttttgtttgcaagcagcagattacgcgcagaaaaaaaggatctcaagaagatcctttgatcttttctacggggtctgacgctcagtggaacgaaaactcacgttaagggattttggtcatgagattatcaaaaaggatcttcacctagatccttttaaattaaaaatgaagttttaaatcaatctaaagtatatatgagtaaacttggtctgacagttaccaatgcttaatcagtgaggcacctatctcagcgatctgtctatttcgttcatccatagttgcctgactccccgtcgtgtagataactacgatacgggagggcttaccatctggccccagtgctgcaatgataccgcgagaaccacgctcaccggctccagatttatcagcaataaaccagccagccggaagggccgagcgcagaagtggtcctgcaactttatccgcctccatccagtctattaattgttgccgggaagctagagtaagtagttcgccagttaatagtttgcgcaacgttgttgccattgctacaggcatcgtggtgtcacgctcgtcgtttggtatggcttcattcagctccggttcccaacgatcaaggcgagttacatgatcccccatgttgtgcaaaaaagcggttagctccttcggtcctccgatcgttgtcagaagtaagttggccgcagtgttatcactcatggttatggcagcactgcataattctcttactgtcatgccatccgtaagatgcttttctgtgactggtgagtactcaaccaagtcattctgagaatagtgtatgcggcgaccgagttgctcttgcccggcgtcaatacgggataataccgcgccacatagcagaactttaaaagtgctcatcattggaaaacgttcttcggggcgaaaactctcaaggatcttaccgctgttgagatccagttcgatgtaacccactcgtgcacccaactgatcttcagcatcttttactttcaccagcgtttctgggtgagcaaaaacaggaaggcaaaatgccgcaaaaaagggaataagggcgacacggaaatgttgaatactcatactcttcctttttcaatattattgaagcatttatcagggttattgtctcatgagcggatacatatttgaatgtatttagaaaaataaacaaataggggttccgcgcacatttccccgaaaagtgccac

SEQ ID NO: 80 - DNA, 3593 bp, Artificial Sequence
  pMA_F14_HLA-B*35:01-6xHis_F15 vector V4.H.8
ctaaattgtaagcgttaatattttgttaaaattcgcgttaaatttttgttaaatcagctcattttttaaccaataggccgaaatcggcaaaatcccttataaatcaaaagaatagaccgagatagggttgagtggccgctacagggcgctcccattcgccattcaggctgcgcaactgttgggaagggcgtttcggtgcgggcctcttcgctattacgccagctggcgaaagggggatgtgctgcaaggcgattaagttgggtaacgccagggttttcccagtcacgacgttgtaaaacgacggccagtgagcgcgacgtaatacgactcactatagggcgaattggcggaaggccgtcaaggccgcatgaattcgctaccgggaagttcctattccgaagttcctattctatcagaagtataggaacttcaggtaccatgcgggtcacggcgccccgaaccgtcctcctgctgctctggggggcagtggccctgaccgagacctgggccggctcccactccatgaggtatttctacaccgccatgtcccggccaggacgcggagagccacgcttcatcgcagtgggctacgtggacgacacccagttcgtgaggttcgacagcgacgccgcgagtccgaggacggagcctcgggcgccatggatagagcaggaggggccggagtattgggaccggaacacacagatcttcaagaccaacacacagacttaccgagagagcctgcggaacctgcgcggctactacaaccagagcgaggccgggtctcacatcatccagaggatgtatggctgcgacctggggcccgacgggcgcctcctccgcgggcatgaccagtccgcctacgacggcaaggattacatcgccctgaacgaggacctgagctcctggaccgcggcggacaccgcggctcagatcacccagcgcaagtgggaggcggcccgtgtggcggagcagctgagagcctacctggagggcctgtgcgtggagtggctccgcagatacctggagaacgggaaggagactcttcagcgcgcagatcctccaaagacacacgtgacccaccaccccgtctctgaccatgaggccaccctgaggtgctgggccctgggcttctaccctgcggagatcacactgacctggcagcgggatggcgaggaccaaactcaggacactgagcttgtggagaccagaccagcaggagatagaaccttccagaagtgggcagctgtggtggtgccttctggagaagagcagagatacacatgccatgtacagcatgaggggctgccgaagcccctcaccctgagatgggagccatcttcccagtccaccatccccatcgtgggcattgttgctggcctggctgtcctagcagttgtggtcatcggagctgtggtcgctactgtgatgtgtaggaggaagagctcaggtggaaaaggagggagctactctcaggctgcgtccagcgacagtgcccagggctctgatgtgtctctcacagctcccgggcatcatcaccatcaccactgactatagtcgtctagacgaagttcctattccgaagttcctattcttataggagtataggaacttcctcgagctgggcctcatgggccttccgctcactgcccgctttccagtcgggaaacctgtcgtgccagctgcattaacatggtcatagctgtttccttgcgtattgggcgctctccgcttcctcgctcactgactcgctgcgctcggtcgttcgggtaaagcctggggtgcctaatgagcaaaaggccagcaaaaggccaggaaccgtaaaaaggccgcgttgctggcgtttttccataggctccgcccccctgacgagcatcacaaaaatcgacgctcaagtcagaggtggcgaaacccgacaggactataaagataccaggcgtttccccctggaagctccctcgtgcgctctcctgttccgaccctgccgcttaccggatacctgtccgcctttctcccttcgggaagcgtggcgctttctcatagctcacgctgtaggtatctcagttcggtgtaggtcgttcgctccaagctgggctgtgtgcacgaaccccccgttcagcccgaccgctgcgccttatccggtaactatcgtcttgagtccaacccggtaagacacgacttatcgccactggcagcagccactggtaacaggattagcagagcgaggtatgtaggcggtgctacagagttcttgaagtggtggcctaactacggctacactagaagaacagtatttggtatctgcgctctgctgaagccagttaccttcggaaaaagagttggtagctcttgatccggcaaacaaaccaccgctggtagcggtggtttttttgtttgcaagcagcagattacgcgcagaaaaaaaggatctcaagaagatcctttgatcttttctacggggtctgacgctcagtggaacgaaaactcacgttaagggattttggtcatgagattatcaaaaaggatcttcacctagatccttttaaattaaaaatgaagttttaaatcaatctaaagtatatatgagtaaacttggtctgacagttaccaatgcttaatcagtgaggcacctatctcagcgatctgtctatttcgttcatccatagttgcctgactccccgtcgtgtagataactacgatacgggagggcttaccatctggccccagtgctgcaatgataccgcgagaaccacgctcaccggctccagatttatcagcaataaaccagccagccggaagggccgagcgcagaagtggtcctgcaactttatccgcctccatccagtctattaattgttgccgggaagctagagtaagtagttcgccagttaatagtttgcgcaacgttgttgccattgctacaggcatcgtggtgtcacgctcgtcgtttggtatggcttcattcagctccggttcccaacgatcaaggcgagttacatgatcccccatgttgtgcaaaaaagcggttagctccttcggtcctccgatcgttgtcagaagtaagttggccgcagtgttatcactcatggttatggcagcactgcataattctcttactgtcatgccatccgtaagatgcttttctgtgactggtgagtactcaaccaagtcattctgagaatagtgtatgcggcgaccgagttgctcttgcccggcgtcaatacgggataataccgcgccacatagcagaactttaaaagtgctcatcattggaaaacgttcttcggggcgaaaactctcaaggatcttaccgctgttgagatccagttcgatgtaacccactcgtgcacccaactgatcttcagcatcttttactttcaccagcgtttctgggtgagcaaaaacaggaaggcaaaatgccgcaaaaaagggaataagggcgacacggaaatgttgaatactcatactcttcctttttcaatattattgaagcatttatcagggttattgtctcatgagcggatacatatttgaatgtatttagaaaaataaacaaataggggttccgcgcacatttccccgaaaagtgccac

SEQ ID NO: 81 - DNA, 3172 bp, Artificial Sequence
  FRT_HCMVpp28-3xMYC_F3 vector V9.E.6
ggcggttcctctacatccggtggatctggatctggagaacaaaagctcatctctgaggaggaccttggggagcagaagctaatcagtgaagaagacctcggagagcagaaattgattagcgaggaggatctttaaagactaggcacgaagttcctattccgaagttcctattcttcaaatagtataggaacttccgctctgaccagctgcattaacatggtcatagctgtttccttgcgtattgggcgctctccgcttcctcgctcactgactcgctgcgctcggtcgttcgggtaaagcctggggtgcctaatgagcaaaaggccagcaaaaggccaggaaccgtaaaaaggccgcgttgctggcgtttttccataggctccgcccccctgacgagcatcacaaaaatcgacgctcaagtcagaggtggcgaaacccgacaggactataaagataccaggcgtttccccctggaagctccctcgtgcgctctcctgttccgaccctgccgcttaccggatacctgtccgcctttctcccttcgggaagcgtggcgctttctcatagctcacgctgtaggtatctcagttcggtgtaggtcgttcgctccaagctgggctgtgtgcacgaaccccccgttcagcccgaccgctgcgccttatccggtaactatcgtcttgagtccaacccggtaagacacgacttatcgccactggcagcagccactggtaacaggattagcagagcgaggtatgtaggcggtgctacagagttcttgaagtggtggcctaactacggctacactagaagaacagtatttggtatctgcgctctgctgaagccagttaccttcggaaaaagagttggtagctcttgatccggcaaacaaaccaccgctggtagcggtggtttttttgtttgcaagcagcagattacgcgcagaaaaaaaggatctcaagaagatcctttgatcttttctacggggtctgacgctcagtggaacgaaaactcacgttaagggattttggtcatgagattatcaaaaaggatcttcacctagatccttttaaattaaaaatgaagttttaaatcaatctaaagtatatatgagtaaacttggtctgacagttaccaatgcttaatcagtgaggcacctatctcagcgatctgtctatttcgttcatccatagttgcctgactccccgtcgtgtagataactacgatacgggagggcttaccatctggccccagtgctgcaatgataccgcgagaaccacgctcaccggctccagatttatcagcaataaaccagccagccggaagggccgagcgcagaagtggtcctgcaactttatccgcctccatccagtctattaattgttgccgggaagctagagtaagtagttcgccagttaatagtttgcgcaacgttgttgccattgctacaggcatcgtggtgtcacgctcgtcgtttggtatggcttcattcagctccggttcccaacgatcaaggcgagttacatgatcccccatgttgtgcaaaaaagcggttagctccttcggtcctccgatcgttgtcagaagtaagttggccgcagtgttatcactcatggttatggcagcactgcataattctcttactgtcatgccatccgtaagatgcttttctgtgactggtgagtactcaaccaagtcattctgagaatagtgtatgcggcgaccgagttgctcttgcccggcgtcaatacgggataataccgcgccacatagcagaactttaaaagtgctcatcattggaaaacgttcttcggggcgaaaactctcaaggatcttaccgctgttgagatccagttcgatgtaacccactcgtgcacccaactgatcttcagcatcttttactttcaccagcgtttctgggtgagcaaaaacaggaaggcaaaatgccgcaaaaaagggaataagggcgacacggaaatgttgaatactcatactcttcctttttcaatattattgaagcatttatcagggttattgtctcatgagcggatacatatttgaatgtatttagaaaaataaacaaataggggttccgcgcacatttccccgaaaagtgccacctaaattgtaagcgttaatattttgttaaaattcgcgttaaatttttgttaaatcagctcattttttaaccaataggccgaaatcggcaaaatcccttataaatcaaaagaatagaccgagatagggttgagtggccgctacagggcgctcccattcgccattcaggctgcgcaactgttgggaagggcgtttcggtgcgggcctcttcgctattacgccagctggcgaaagggggatgtgctgcaaggcgattaagttgggtaacgccagggttttcccagtcacgacgttgtaaaacgacggccagtgagcgcgacgtaatacgactcactatagggcgaattggcggaaggccgtcaaggccgcatgaattcgctaccgggagttggtaggtaagtatcaaggttacaagacaggtttaaggaggaagttcctattccgaagttcctattctctagaaagtataggaacttcgactctcaccatgggtgccgaactctgcaaacgaatatgttgtgagttcggtaccacgtccggtgagcccctgaaagatgctctgggtcgccaggtgtctctacgctcctacgacaacatccctccgacttcctcctcggacgaaggggaggacgatgacgacggggaggatgacgataacgaggagcggcaacagaagctgcggctctgcggtagtggctgcggaggaaacgacagtagcagtggcagccaccgagaggccacccacgacggccctaagaagaacgctgtgcgctcgacgtttcgcgaggacaaggctccgaaaccgagcaagcagtccaagaagaaaaagaaaccctcaaagcatcaccaccatcagcaaagctccattatgcaggagacggacgacttagacgaagaggacacctcaatttacctgtcccctccccctgttccaccagttcaggtggtggctaagcgactgccgcgtcccgacacacccaggactccgcgccagaagaagatttcacaacgtccacccacacccgggaccaaaaagcccgctgcctccttgcccttt

SEQ ID NO: 82 - DNA, 3900 bp, Artificial Sequence
  FRT_HCMVpp52-3xMYC_F3 vector V9.E.7
ggcggttcctctacatccggtggatctggatctggagaacaaaagctcatctctgaggaggaccttggggagcagaagctaatcagtgaagaagacctcggagagcagaaattgattagcgaggaggatctttaaagactaggcacgaagttcctattccgaagttcctattcttcaaatagtataggaacttccgctctgaccagctgcattaacatggtcatagctgtttccttgcgtattgggcgctctccgcttcctcgctcactgactcgctgcgctcggtcgttcgggtaaagcctggggtgcctaatgagcaaaaggccagcaaaaggccaggaaccgtaaaaaggccgcgttgctggcgtttttccataggctccgcccccctgacgagcatcacaaaaatcgacgctcaagtcagaggtggcgaaacccgacaggactataaagataccaggcgtttccccctggaagctccctcgtgcgctctcctgttccgaccctgccgcttaccggatacctgtccgcctttctcccttcgggaagcgtggcgctttctcatagctcacgctgtaggtatctcagttcggtgtaggtcgttcgctccaagctgggctgtgtgcacgaaccccccgttcagcccgaccgctgcgccttatccggtaactatcgtcttgagtccaacccggtaagacacgacttatcgccactggcagcagccactggtaacaggattagcagagcgaggtatgtaggcggtgctacagagttcttgaagtggtggcctaactacggctacactagaagaacagtatttggtatctgcgctctgctgaagccagttaccttcggaaaaagagttggtagctcttgatccggcaaacaaaccaccgctggtagcggtggtttttttgtttgcaagcagcagattacgcgcagaaaaaaaggatctcaagaagatcctttgatcttttctacggggtctgacgctcagtggaacgaaaactcacgttaagggattttggtcatgagattatcaaaaaggatcttcacctagatccttttaaattaaaaatgaagttttaaatcaatctaaagtatatatgagtaaacttggtctgacagttaccaatgcttaatcagtgaggcacctatctcagcgatctgtctatttcgttcatccatagttgcctgactccccgtcgtgtagataactacgatacgggagggcttaccatctggccccagtgctgcaatgataccgcgagaaccacgctcaccggctccagatttatcagcaataaaccagccagccggaagggccgagcgcagaagtggtcctgcaactttatccgcctccatccagtctattaattgttgccgggaagctagagtaagtagttcgccagttaatagtttgcgcaacgttgttgccattgctacaggcatcgtggtgtcacgctcgtcgtttggtatggcttcattcagctccggttcccaacgatcaaggcgagttacatgatcccccatgttgtgcaaaaaagcggttagctccttcggtcctccgatcgttgtcagaagtaagttggccgcagtgttatcactcatggttatggcagcactgcataattctcttactgtcatgccatccgtaagatgcttttctgtgactggtgagtactcaaccaagtcattctgagaatagtgtatgcggcgaccgagttgctcttgcccggcgtcaatacgggataataccgcgccacatagcagaactttaaaagtgctcatcattggaaaacgttcttcggggcgaaaactctcaaggatcttaccgctgttgagatccagttcgatgtaacccactcgtgcacccaactgatcttcagcatcttttactttcaccagcgtttctgggtgagcaaaaacaggaaggcaaaatgccgcaaaaaagggaataagggcgacacggaaatgttgaatactcatactcttcctttttcaatattattgaagcatttatcagggttattgtctcatgagcggatacatatttgaatgtatttagaaaaataaacaaataggggttccgcgcacatttccccgaaaagtgccacctaaattgtaagcgttaatattttgttaaaattcgcgttaaatttttgttaaatcagctcattttttaaccaataggccgaaatcggcaaaatcccttataaatcaaaagaatagaccgagatagggttgagtggccgctacagggcgctcccattcgccattcaggctgcgcaactgttgggaagggcgtttcggtgcgggcctcttcgctattacgccagctggcgaaagggggatgtgctgcaaggcgattaagttgggtaacgccagggttttcccagtcacgacgttgtaaaacgacggccagtgagcgcgacgtaatacgactcactatagggcgaattggcggaaggccgtcaaggccgcatgaattcgctaccgggagttggtaggtaagtatcaaggttacaagacaggtttaaggaggaagttcctattccgaagttcctattctctagaaagtataggaacttcgactctaccaccatggatcgcaagacgcgcctctcggagccgccgacgctggcgctgcggctgaagccgtacaagacggctatccagcagctgcgatctgtgatccgtgcgctcaaggagaacaccacggttaccttcttgcccacaccgtcgcttatcttgcaaacggtacgcagtcactgcgtgtcaaagatcacttttaacagctcatgcctctacatcactgacaagtcgtttcagcccaagaccattaacaattccacgcctctgctgggtaacttcatgtacctgacttccagcaaggacctgaccaagttctacgtgcaggacatctcggacctgtcggccaagatctccatgtgcgcacccgatttcaatatggagttcagctcggcctgcgtgcacggccaagacattgtgcgcgaaagcgagaattcggccgtgcacgtggatctagatttcggcgtggtggccgacctgcttaagtggatcgggccgcatacccgcgtcaagcgtaacgtgaagaaagcgccctgccctacgggcaccgtgcagattctggtgcacgccggtccaccggccatcaagttcatcctgaccaacggcagcgagctggaattcacagccaataaccgcgtcagtttccacggcgtgaaaaacatgcgtatcaacgtgcagctgaagaacttctaccagacgctgctcaattgcgccgtcaccaaactgccgtgcacgttgcgtatagttacggagcacgacacgctgttgtacgtggccagccgcaacggtctgttcgccgtggagaattttctcaccgaggaacctttccagcgtggcgatcccttcgacaagaattacgtcgggaacagcggcaaatcgcgtggcggaggcggtggtagcggcagcctctcttcgctggctaatgccggcggtctgcacgacgacggtccgggtctggacaacgatatcatgaacgagcccatgggtctcggcggactgggaggtggcggaggagggggaggcaagaagcacgaccgcggaggtggcggtggttccggtacgcggaaaatgagcagcggtggcggaggtggagatcacgaccacggtctttcctccaaggaaaaatacgagcagcacaagatcaccagctacctgacgtccaaaggtggatcgggaggagggggtggaggcggaggtggaggtttggatcgcaactccggcaattacttcaacgacgcgaaagaggagagcgacagcgaggattctgtaacgttcgagttcgtccctaacaccaagaagcaaaagtgc

SEQ ID NO: 83 - DNA, 4286 bp, Artificial Sequence
  FRT_HCMVpp52-3xMYC_F3 vector V9.E.8
ggcggttcctctacatccggtggatctggatctggagaacaaaagctcatctctgaggaggaccttggggagcagaagctaatcagtgaagaagacctcggagagcagaaattgattagcgaggaggatctttaaagactaggcacgaagttcctattccgaagttcctattcttcaaatagtataggaacttccgctctgaccagctgcattaacatggtcatagctgtttccttgcgtattgggcgctctccgcttcctcgctcactgactcgctgcgctcggtcgttcgggtaaagcctggggtgcctaatgagcaaaaggccagcaaaaggccaggaaccgtaaaaaggccgcgttgctggcgtttttccataggctccgcccccctgacgagcatcacaaaaatcgacgctcaagtcagaggtggcgaaacccgacaggactataaagataccaggcgtttccccctggaagctccctcgtgcgctctcctgttccgaccctgccgcttaccggatacctgtccgcctttctcccttcgggaagcgtggcgctttctcatagctcacgctgtaggtatctcagttcggtgtaggtcgttcgctccaagctgggctgtgtgcacgaaccccccgttcagcccgaccgctgcgccttatccggtaactatcgtcttgagtccaacccggtaagacacgacttatcgccactggcagcagccactggtaacaggattagcagagcgaggtatgtaggcggtgctacagagttcttgaagtggtggcctaactacggctacactagaagaacagtatttggtatctgcgctctgctgaagccagttaccttcggaaaaagagttggtagctcttgatccggcaaacaaaccaccgctggtagcggtggtttttttgtttgcaagcagcagattacgcgcagaaaaaaaggatctcaagaagatcctttgatcttttctacggggtctgacgctcagtggaacgaaaactcacgttaagggattttggtcatgagattatcaaaaaggatcttcacctagatccttttaaattaaaaatgaagttttaaatcaatctaaagtatatatgagtaaacttggtctgacagttaccaatgcttaatcagtgaggcacctatctcagcgatctgtctatttcgttcatccatagttgcctgactccccgtcgtgtagataactacgatacgggagggcttaccatctggccccagtgctgcaatgataccgcgagaaccacgctcaccggctccagatttatcagcaataaaccagccagccggaagggccgagcgcagaagtggtcctgcaactttatccgcctccatccagtctattaattgttgccgggaagctagagtaagtagttcgccagttaatagtttgcgcaacgttgttgccattgctacaggcatcgtggtgtcacgctcgtcgtttggtatggcttcattcagctccggttcccaacgatcaaggcgagttacatgatcccccatgttgtgcaaaaaagcggttagctccttcggtcctccgatcgttgtcagaagtaagttggccgcagtgttatcactcatggttatggcagcactgcataattctcttactgtcatgccatccgtaagatgcttttctgtgactggtgagtactcaaccaagtcattctgagaatagtgtatgcggcgaccgagttgctcttgcccggcgtcaatacgggataataccgcgccacatagcagaactttaaaagtgctcatcattggaaaacgttcttcggggcgaaaactctcaaggatcttaccgctgttgagatccagttcgatgtaacccactcgtgcacccaactgatcttcagcatcttttactttcaccagcgtttctgggtgagcaaaaacaggaaggcaaaatgccgcaaaaaagggaataagggcgacacggaaatgttgaatactcatactcttcctttttcaatattattgaagcatttatcagggttattgtctcatgagcggatacatatttgaatgtatttagaaaaataaacaaataggggttccgcgcacatttccccgaaaagtgccacctaaattgtaagcgttaatattttgttaaaattcgcgttaaatttttgttaaatcagctcattttttaaccaataggccgaaatcggcaaaatcccttataaatcaaaagaatagaccgagatagggttgagtggccgctacagggcgctcccattcgccattcaggctgcgcaactgttgggaagggcgtttcggtgcgggcctcttcgctattacgccagctggcgaaagggggatgtgctgcaaggcgattaagttgggtaacgccagggttttcccagtcacgacgttgtaaaacgacggccagtgagcgcgacgtaatacgactcactatagggcgaattggcggaaggccgtcaaggccgcatgaattcgctaccgggagttggtaggtaagtatcaaggttacaagacaggtttaaggaggaagttcctattccgaagttcctattctctagaaagtataggaacttcgactctcaggtaccatggagtcgcgcggtcgccgttgtcccgaaatgatatccgtactgggtcccatttcggggcacgtgctgaaagccgtgtttagtcgcggcgatacgccggtgctgccgcacgagacgcgactcctgcagacgggtatccacgtacgcgtgagccagccctcgctgatcttggtatcgcagtacacgcccgactcgacgccatgccaccgcggcgacaatcagctgcaggtgcagcacacgtactttacgggcagcgaggtggagaacgtgtcggtcaacgtgcacaaccccacgggccgaagcatctgccccagccaggagcccatgtcgatctatgtgtacgcgctgccgctcaagatgctgaacatccccagcatcaacgtgcaccactacccgtcggcggccgagcgcaaacaccgacacctgcccgtagctgacgctgtgattcacgcgtcgggcaagcagatgtggcaggcgcgtctcacggtctcgggactggcctggacgcgtcagcagaaccagtggaaagagcccgacgtctactacacgtcagcgttcgtgtttcccaccaaggacgtggcactgcggcacgtggtgtgcgcgcacgagctggtttgctccatggagaacacgcgcgcaaccaagatgcaggtgataggtgaccagtacgtcaaggtgtacctggagtccttctgcgaggacgtgccctccggcaagctctttatgcacgtcacgctgggctctgacgtggaagaggacctgacgatgacccgcaacccgcaacccttcatgcgcccccacgagcgcaacggctttacggtgttgtgtcccaaaaatatgataatcaaaccgggcaagatctcgcacatcatgctggatgtggcttttacctcacacgagcattttgggctgctgtgtcccaagagcatcccgggcctgagcatctcaggtaacctgttgatgaacgggcagcagatcttcctggaggtacaagccatacgcgagaccgtggaactgcgtcagtacgatcccgtggctgcgctcttctttttcgatatcgacttgctgctgcagcgcgggcctcagtacagcgagcaccccaccttcaccagccagtatcgcatccagggcaagcttgagtaccgacacacctgggaccggcacgacgagggtgccgcccagggcgacgacgacgtctggaccagcggatcggactccgacgaagaactcgtaaccaccgagcgcaagacgccccgcgtcaccggcggcggcgccatggcgggcgcctccacttccgcgggccgcaaacgcaaatcagcatcctcggcgacggcgtgcacgtcgggcgttatgacacgcggccgccttaaggccgagtccaccgtcgcgcccgaagaggacaccgacgaggattccgacaacgaaatccacaatccggccgtgttcacctggccgccctggcaggccggcatcctggcccgcaacctggtgcccatggtggctacggttcagggtcagaatctgaagtaccaggagttcttctgggacgccaacgacatctaccgcatcttcgccgaattggaaggcgtatggcagcccgctgcgcaacccaaacgtcgccgccaccggcaagacgccttgcccgggccatgcatcgcctcgacgcccaaaaagcaccga

SEQ ID NO: 84 - DNA, 10428 bp, Artificial Sequence
  SpCas9-2A-GFP Vector V1.A.8
gacggatcgggagatctcccgatcccctatggtgcactctcagtacaatctgctctgatgccgcatagttaagccagtatctgctccctgcttgtgtgttggaggtcgctgagtagtgcgcgagcaaaatttaagctacaacaaggcaaggcttgaccgacaattgcatgaagaatctgcttagggttaggcgttttgcgctgcttcgcgatgtacgggccagatatacgcgttgacattgattattgactagttattaatagtaatcaattacggggtcattagttcatagcccatatatggagttccgcgttacataacttacggtaaatggcccgcctggctgaccgcccaacgacccccgcccattgacgtcaataatgacgtatgttcccatagtaacgccaatagggactttccattgacgtcaatgggtggagtatttacggtaaactgcccacttggcagtacatcaagtgtatcatatgccaagtacgccccctattgacgtcaatgacggtaaatggcccgcctggcattatgcccagtacatgaccttatgggactttcctacttggcagtacatctacgtattagtcatcgctattaccatggtgatgcggttttggcagtacatcaatgggcgtggatagcggtttgactcacggggatttccaagtctccaccccattgacgtcaatgggagtttgttttggcaccaaaatcaacgggactttccaaaatgtcgtaacaactccgccccattgacgcaaatgggcggtaggcgtgtacggtgggaggtctatataagcagagctctctggctaactagagaacccactgcttactggcttatcgaaattaatacgactcactatagggagacccaagctggctagcgtttaaacttaagcttggtaccgccaccatggactataaggaccacgacggagactacaaggatcatgatattgattacaaagacgatgacgataagatggccccaaagaagaagcggaaggtcggtatccacggagtcccagcagccgacaagaagtacagcatcggcctggacatcggcaccaactctgtgggctgggccgtgatcaccgacgagtacaaggtgcccagcaagaaattcaaggtgctgggcaacaccgaccggcacagcatcaagaagaacctgatcggagccctgctgttcgacagcggcgaaacagccgaggccacccggctgaagagaaccgccagaagaagatacaccagacggaagaaccggatctgctatctgcaagagatcttcagcaacgagatggccaaggtggacgacagcttcttccacagactggaagagtccttcctggtggaagaggataagaagcacgagcggcaccccatcttcggcaacatcgtggacgaggtggcctaccacgagaagtaccccaccatctaccacctgagaaagaaactggtggacagcaccgacaaggccgacctgcggctgatctatctggccctggcccacatgatcaagttccggggccacttcctgatcgagggcgacctgaaccccgacaacagcgacgtggacaagctgttcatccagctggtgcagacctacaaccagctgttcgaggaaaaccccatcaacgccagcggcgtggacgccaaggccatcctgtctgccagactgagcaagagcagacggctggaaaatctgatcgcccagctgcccggcgagaagaagaatggcctgttcggaaacctgattgccctgagcctgggcctgacccccaacttcaagagcaacttcgacctggccgaggatgccaaactgcagctgagcaaggacacctacgacgacgacctggacaacctgctggcccagatcggcgaccagtacgccgacctgtttctggccgccaagaacctgtccgacgccatcctgctgagcgacatcctgagagtgaacaccgagatcaccaaggcccccctgagcgcctctatgatcaagagatacgacgagcaccaccaggacctgaccctgctgaaagctctcgtgcggcagcagctgcctgagaagtacaaagagattttcttcgaccagagcaagaacggctacgccggctacattgacggcggagccagccaggaagagttctacaagttcatcaagcccatcctggaaaagatggacggcaccgaggaactgctcgtgaagctgaacagagaggacctgctgcggaagcagcggaccttcgacaacggcagcatcccccaccagatccacctgggagagctgcacgccattctgcggcggcaggaagatttttacccattcctgaaggacaaccgggaaaagatcgagaagatcctgaccttccgcatcccctactacgtgggccctctggccaggggaaacagcagattcgcctggatgaccagaaagagcgaggaaaccatcaccccctggaacttcgaggaagtggtggacaagggcgcttccgcccagagcttcatcgagcggatgaccaacttcgataagaacctgcccaacgagaaggtgctgcccaagcacagcctgctgtacgagtacttcaccgtgtataacgagctgaccaaagtgaaatacgtgaccgagggaatgagaaagcccgccttcctgagcggcgagcagaaaaaggccatcgtggacctgctgttcaagaccaaccggaaagtgaccgtgaagcagctgaaagaggactacttcaagaaaatcgagtgcttcgactccgtggaaatctccggcgtggaagatcggttcaacgcctccctgggcacataccacgatctgctgaaaattatcaaggacaaggacttcctggacaatgaggaaaacgaggacattctggaagatatcgtgctgaccctgacactgtttgaggacagagagatgatcgaggaacggctgaaaacctatgcccacctgttcgacgacaaagtgatgaagcagctgaagcggcggagatacaccggctggggcaggctgagccggaagctgatcaacggcatccgggacaagcagtccggcaagacaatcctggatttcctgaagtccgacggcttcgccaacagaaacttcatgcagctgatccacgacgacagcctgacctttaaagaggacatccagaaagcccaggtgtccggccagggcgatagcctgcacgagcacattgccaatctggccggcagccccgccattaagaagggcatcctgcagacagtgaaggtggtggacgagctcgtgaaagtgatgggccggcacaagcccgagaacatcgtgatcgaaatggccagagagaaccagaccacccagaagggacagaagaacagccgcgagagaatgaagcggatcgaagagggcatcaaagagctgggcagccagatcctgaaagaacaccccgtggaaaacacccagctgcagaacgagaagctgtacctgtactacctgcagaatgggcgggatatgtacgtggaccaggaactggacatcaaccggctgtccgactacgatgtggaccatatcgtgcctcagagctttctgaaggacgactccatcgacaacaaggtgctgaccagaagcgacaagaaccggggcaagagcgacaacgtgccctccgaagaggtcgtgaagaagatgaagaactactggcggcagctgctgaacgccaagctgattacccagagaaagttcgacaatctgaccaaggccgagagaggcggcctgagcgaactggataaggccggcttcatcaagagacagctggtggaaacccggcagatcacaaagcacgtggcacagatcctggactcccggatgaacactaagtacgacgagaatgacaagctgatccgggaagtgaaagtgatcaccctgaagtccaagctggtgtccgatttccggaaggatttccagttttacaaagtgcgcgagatcaacaactaccaccacgcccacgacgcctacctgaacgccgtcgtgggaaccgccctgatcaaaaagtaccctaagctggaaagcgagttcgtgtacggcgactacaaggtgtacgacgtgcggaagatgatcgccaagagcgagcaggaaatcggcaaggctaccgccaagtacttcttctacagcaacatcatgaactttttcaagaccgagattaccctggccaacggcgagatccggaagcggcctctgatcgagacaaacggcgaaaccggggagatcgtgtgggataagggccgggattttgccaccgtgcggaaagtgctgagcatgccccaagtgaatatcgtgaaaaagaccgaggtgcagacaggcggcttcagcaaagagtctatcctgcccaagaggaacagcgataagctgatcgccagaaagaaggactgggaccctaagaagtacggcggcttcgacagccccaccgtggcctattctgtgctggtggtggccaaagtggaaaagggcaagtccaagaaactgaagagtgtgaaagagctgctggggatcaccatcatggaaagaagcagcttcgagaagaatcccatcgactttctggaagccaagggctacaaagaagtgaaaaaggacctgatcatcaagctgcctaagtactccctgttcgagctggaaaacggccggaagagaatgctggcctctgccggcgaactgcagaagggaaacgaactggccctgccctccaaatatgtgaacttcctgtacctggccagccactatgagaagctgaagggctcccccgaggataatgagcagaaacagctgtttgtggaacagcacaagcactacctggacgagatcatcgagcagatcagcgagttctccaagagagtgatcctggccgacgctaatctggacaaagtgctgtccgcctacaacaagcaccgggataagcccatcagagagcaggccgagaatatcatccacctgtttaccctgaccaatctgggagcccctgccgccttcaagtactttgacaccaccatcgaccggaagaggtacaccagcaccaaagaggtgctggacgccaccctgatccaccagagcatcaccggcctgtacgagacacggatcgacctgtctcagctgggaggcgacaaaaggccggcggccacgaaaaaggccggccaggcaaaaaagaaaaaggaattcggcagtggagagggcagaggaagtctgctaacatgcggtgacgtcgaggagaatcctggcccagtgagcaagggcgaggagctgttcaccggggtggtgcccatcctggtcgagctggacggcgacgtaaacggccacaagttcagcgtgtccggcgagggcgagggcgatgccacctacggcaagctgaccctgaagttcatctgcaccaccggcaagctgcccgtgccctggcccaccctcgtgaccaccctgacctacggcgtgcagtgcttcagccgctaccccgaccacatgaagcagcacgacttcttcaagtccgccatgcccgaaggctacgtccaggagcgcaccatcttcttcaaggacgacggcaactacaagacccgcgccgaggtgaagttcgagggcgacaccctggtgaaccgcatcgagctgaagggcatcgacttcaaggaggacggcaacatcctggggcacaagctggagtacaactacaacagccacaacgtctatatcatggccgacaagcagaagaacggcatcaaggtgaacttcaagatccgccacaacatcgaggacggcagcgtgcagctcgccgaccactaccagcagaacacccccatcggcgacggccccgtgctgctgcccgacaaccactacctgagcacccagtccgccctgagcaaagaccccaacgagaagcgcgatcacatggtcctgctggagttcgtgaccgccgccgggatcactctcggcatggacgagctgtacaaggaattctaacgctagagggcccgtttaaacccgctgatcagcctcgactgtgccttctagttgccagccatctgttgtttgcccctcccccgtgccttccttgaccctggaaggtgccactcccactgtcctttcctaataaaatgaggaaattgcatcgcattgtctgagtaggtgtcattctattctggggggtggggtggggcaggacagcaagggggaggattgggaagacaatagcaggcatgctggggatgcggtgggctctatggcttctgaggcggaaagaaccagctggggctctagggggtatccccacgcgccctgtagcggcgcattaagcgcggcgggtgtggtggttacgcgcagcgtgaccgctacacttgccagcgccctagcgcccgctcctttcgctttcttcccttcctttctcgccacgttcgccggctttccccgtcaagctctaaatcgggggctccctttagggttccgatttagtgctttacggcacctcgaccccaaaaaacttgattagggtgatggttcacgtagtgggccatcgccctgatagacggtttttcgccctttgacgttggagtccacgttctttaatagtggactcttgttccaaactggaacaacactcaaccctatctcggtctattcttttgatttataagggattttgccgatttcggcctattggttaaaaaatgagctgatttaacaaaaatttaacgcgaattaattctgtggaatgtgtgtcagttagggtgtggaaagtccccaggctccccagcaggcagaagtatgcaaagcatgcatctcaattagtcagcaaccaggtgtggaaagtccccaggctccccagcaggcagaagtatgcaaagcatgcatctcaattagtcagcaaccatagtcccgcccctaactccgcccatcccgcccctaactccgcccagttccgcccattctccgccccatggctgactaattttttttatttatgcagaggccgaggccgcctctgcctctgagctattccagaagtagtgaggaggcttttttggaggcctaggcttttgcaaaaagctcccgggagcttgtatatccattttcggatctgatcaagagacaggatgaggatcgtttcgcatgattgaacaagatggattgcacgcaggttctccggccgcttgggtggagaggctattcggctatgactgggcacaacagacaatcggctgctctgatgccgccgtgttccggctgtcagcgcaggggcgcccggttctttttgtcaagaccgacctgtccggtgccctgaatgaactgcaggacgaggcagcgcggctatcgtggctggccacgacgggcgttccttgcgcagctgtgctcgacgttgtcactgaagcgggaagggactggctgctattgggcgaagtgccggggcaggatctcctgtcatctcaccttgctcctgccgagaaagtatccatcatggctgatgcaatgcggcggctgcatacgcttgatccggctacctgcccattcgaccaccaagcgaaacatcgcatcgagcgagcacgtactcggatggaagccggtcttgtcgatcaggatgatctggacgaagagcatcaggggctcgcgccagccgaactgttcgccaggctcaaggcgcgcatgcccgacggcgaggatctcgtcgtgacccatggcgatgcctgcttgccgaatatcatggtggaaaatggccgcttttctggattcatcgactgtggccggctgggtgtggcggaccgctatcaggacatagcgttggctacccgtgatattgctgaagagcttggcggcgaatgggctgaccgcttcctcgtgctttacggtatcgccgctcccgattcgcagcgcatcgccttctatcgccttcttgacgagttcttctgagcgggactctggggttcgaaatgaccgaccaagcgacgcccaacctgccatcacgagatttcgattccaccgccgccttctatgaaaggttgggcttcggaatcgttttccgggacgccggctggatgatcctccagcgcggggatctcatgctggagttcttcgcccaccccaacttgtttattgcagcttataatggttacaaataaagcaatagcatcacaaatttcacaaataaagcatttttttcactgcattctagttgtggtttgtccaaactcatcaatgtatcttatcatgtctgtataccgtcgacctctagctagagcttggcgtaatcatggtcatagctgtttcctgtgtgaaattgttatccgctcacaattccacacaacatacgagccggaagcataaagtgtaaagcctggggtgcctaatgagtgagctaactcacattaattgcgttgcgctcactgcccgctttccagtcgggaaacctgtcgtgccagctgcattaatgaatcggccaacgcgcggggagaggcggtttgcgtattgggcgctcttccgcttcctcgctcactgactcgctgcgctcggtcgttcggctgcggcgagcggtatcagctcactcaaaggcggtaatacggttatccacagaatcaggggataacgcaggaaagaacatgtgagcaaaaggccagcaaaaggccaggaaccgtaaaaaggccgcgttgctggcgtttttccataggctccgcccccctgacgagcatcacaaaaatcgacgctcaagtcagaggtggcgaaacccgacaggactataaagataccaggcgtttccccctggaagctccctcgtgcgctctcctgttccgaccctgccgcttaccggatacctgtccgcctttctcccttcgggaagcgtggcgctttctcatagctcacgctgtaggtatctcagttcggtgtaggtcgttcgctccaagctgggctgtgtgcacgaaccccccgttcagcccgaccgctgcgccttatccggtaactatcgtcttgagtccaacccggtaagacacgacttatcgccactggcagcagccactggtaacaggattagcagagcgaggtatgtaggcggtgctacagagttcttgaagtggtggcctaactacggctacactagaagaacagtatttggtatctgcgctctgctgaagccagttaccttcggaaaaagagttggtagctcttgatccggcaaacaaaccaccgctggtagcggtttttttgtttgcaagcagcagattacgcgcagaaaaaaaggatctcaagaagatcctttgatcttttctacggggtctgacgctcagtggaacgaaaactcacgttaagggattttggtcatgagattatcaaaaaggatcttcacctagatccttttaaattaaaaatgaagttttaaatcaatctaaagtatatatgagtaaacttggtctgacagttaccaatgcttaatcagtgaggcacctatctcagcgatctgtctatttcgttcatccatagttgcctgactccccgtcgtgtagataactacgatacgggagggcttaccatctggccccagtgctgcaatgataccgcgagacccacgctcaccggctccagatttatcagcaataaaccagccagccggaagggccgagcgcagaagtggtcctgcaactttatccgcctccatccagtctattaattgttgccgggaagctagagtaagtagttcgccagttaatagtttgcgcaacgttgttgccattgctacaggcatcgtggtgtcacgctcgtcgtttggtatggcttcattcagctccggttcccaacgatcaaggcgagttacatgatcccccatgttgtgcaaaaaagcggttagctccttcggtcctccgatcgttgtcagaagtaagttggccgcagtgttatcactcatggttatggcagcactgcataattctcttactgtcatgccatccgtaagatgcttttctgtgactggtgagtactcaaccaagtcattctgagaatagtgtatgcggcgaccgagttgctcttgcccggcgtcaatacgggataataccgcgccacatagcagaactttaaaagtgctcatcattggaaaacgttcttcggggcgaaaactctcaaggatcttaccgctgttgagatccagttcgatgtaacccactcgtgcacccaactgatcttcagcatcttttactttcaccagcgtttctgggtgagcaaaaacaggaaggcaaaatgccgcaaaaaagggaataagggcgacacggaaatgttgaatactcatactcttcctttttcaatattattgaagcatttatcagggttattgtctcatgagcggatacatatttgaatgtatttagaaaaataaacaaataggggttccgcgcacatttccccgaaaagtgccacctgacgtc

SEQ ID NO: 85 - DNA, 2762 bp, Artificial Sequence
  HLA-A-sg-sp-opti1 vector V2.A.1
ctaaattgtaagcgttaatattttgttaaaattcgcgttaaatttttgttaaatcagctcattttttaaccaataggccgaaatcggcaaaatcccttataaatcaaaagaatagaccgagatagggttgagtggccgctacagggcgctcccattcgccattcaggctgcgcaactgttgggaagggcgtttcggtgcgggcctcttcgctattacgccagctggcgaaagggggatgtgctgcaaggcgattaagttgggtaacgccagggttttcccagtcacgacgttgtaaaacgacggccagtgagcgcgacgtaatacgactcactatagggcgaattggcggaaggccgtcaaggccgcatggatccaaggtcgggcaggaagagggcctatttcccatgattccttcatatttgcatatacgatacaaggctgttagagagataattagaattaatttgactgtaaacacaaagatattagtacaaaatacgtgacgtagaaagtaataatttcttgggtagtttgcagttttaaaattatgttttaaaatggactatcatatgcttaccgtaacttgaaagtatttcgatttcttggctttatatatcttgtggaaaggacgaaacaccgagggttcggggcgccatgagtttaagagctatgctggaaacagcatagcaagtttaaataaggctagtccgttatcaacttgaaaaagtggcaccgagtcggtgctttttttcagacatccatagatctagctcgagttttttttctagactgggcctcatgggccttccgctcactgcccgctttccagtcgggaaacctgtcgtgccagctgcattaacatggtcatagctgtttccttgcgtattgggcgctctccgcttcctcgctcactgactcgctgcgctcggtcgttcgggtaaagcctggggtgcctaatgagcaaaaggccagcaaaaggccaggaaccgtaaaaaggccgcgttgctggcgtttttccataggctccgcccccctgacgagcatcacaaaaatcgacgctcaagtcagaggtggcgaaacccgacaggactataaagataccaggcgtttccccctggaagctccctcgtgcgctctcctgttccgaccctgccgcttaccggatacctgtccgcctttctcccttcgggaagcgtggcgctttctcatagctcacgctgtaggtatctcagttcggtgtaggtcgttcgctccaagctgggctgtgtgcacgaaccccccgttcagcccgaccgctgcgccttatccggtaactatcgtcttgagtccaacccggtaagacacgacttatcgccactggcagcagccactggtaacaggattagcagagcgaggtatgtaggcggtgctacagagttcttgaagtggtggcctaactacggctacactagaagaacagtatttggtatctgcgctctgctgaagccagttaccttcggaaaaagagttggtagctcttgatccggcaaacaaaccaccgctggtagcggtggtttttttgtttgcaagcagcagattacgcgcagaaaaaaaggatctcaagaagatcctttgatcttttctacggggtctgacgctcagtggaacgaaaactcacgttaagggattttggtcatgagattatcaaaaaggatcttcacctagatccttttaaattaaaaatgaagttttaaatcaatctaaagtatatatgagtaaacttggtctgacagttaccaatgcttaatcagtgaggcacctatctcagcgatctgtctatttcgttcatccatagttgcctgactccccgtcgtgtagataactacgatacgggagggcttaccatctggccccagtgctgcaatgataccgcgagaaccacgctcaccggctccagatttatcagcaataaaccagccagccggaagggccgagcgcagaagtggtcctgcaactttatccgcctccatccagtctattaattgttgccgggaagctagagtaagtagttcgccagttaatagtttgcgcaacgttgttgccattgctacaggcatcgtggtgtcacgctcgtcgtttggtatggcttcattcagctccggttcccaacgatcaaggcgagttacatgatcccccatgttgtgcaaaaaagcggttagctccttcggtcctccgatcgttgtcagaagtaagttggccgcagtgttatcactcatggttatggcagcactgcataattctcttactgtcatgccatccgtaagatgcttttctgtgactggtgagtactcaaccaagtcattctgagaatagtgtatgcggcgaccgagttgctcttgcccggcgtcaatacgggataataccgcgccacatagcagaactttaaaagtgctcatcattggaaaacgttcttcggggcgaaaactctcaaggatcttaccgctgttgagatccagttcgatgtaacccactcgtgcacccaactgatcttcagcatcttttactttcaccagcgtttctgggtgagcaaaaacaggaaggcaaaatgccgcaaaaaagggaataagggcgacacggaaatgttgaatactcatactcttcctttttcaatattattgaagcatttatcagggttattgtctcatgagcggatacatatttgaatgtatttagaaaaataaacaaataggggttccgcgcacatttccccgaaaagtgccac

SEQ ID NO: 86 - DNA, 2762 bp, Artificial Sequence
  HLA-B-sg-sp-3 vector V2.A.7
ctaaattgtaagcgttaatattttgttaaaattcgcgttaaatttttgttaaatcagctcattttttaaccaataggccgaaatcggcaaaatcccttataaatcaaaagaatagaccgagatagggttgagtggccgctacagggcgctcccattcgccattcaggctgcgcaactgttgggaagggcgtttcggtgcgggcctcttcgctattacgccagctggcgaaagggggatgtgctgcaaggcgattaagttgggtaacgccagggttttcccagtcacgacgttgtaaaacgacggccagtgagcgcgacgtaatacgactcactatagggcgaattggcggaaggccgtcaaggccgcatggatccaaggtcgggcaggaagagggcctatttcccatgattccttcatatttgcatatacgatacaaggctgttagagagataattagaattaatttgactgtaaacacaaagatattagtacaaaatacgtgacgtagaaagtaataatttcttgggtagtttgcagttttaaaattatgttttaaaatggactatcatatgcttaccgtaacttgaaagtatttcgatttcttggctttatatatcttgtggaaaggacgaaacaccgtagaaatacctcatggagtgtttaagagctatgctggaaacagcatagcaagtttaaataaggctagtccgttatcaacttgaaaaagtggcaccgagtcggtgctttttttcagacatccatagatctagctcgagttttttttctagactgggcctcatgggccttccgctcactgcccgctttccagtcgggaaacctgtcgtgccagctgcattaacatggtcatagctgtttccttgcgtattgggcgctctccgcttcctcgctcactgactcgctgcgctcggtcgttcgggtaaagcctggggtgcctaatgagcaaaaggccagcaaaaggccaggaaccgtaaaaaggccgcgttgctggcgtttttccataggctccgcccccctgacgagcatcacaaaaatcgacgctcaagtcagaggtggcgaaacccgacaggactataaagataccaggcgtttccccctggaagctccctcgtgcgctctcctgttccgaccctgccgcttaccggatacctgtccgcctttctcccttcgggaagcgtggcgctttctcatagctcacgctgtaggtatctcagttcggtgtaggtcgttcgctccaagctgggctgtgtgcacgaaccccccgttcagcccgaccgctgcgccttatccggtaactatcgtcttgagtccaacccggtaagacacgacttatcgccactggcagcagccactggtaacaggattagcagagcgaggtatgtaggcggtgctacagagttcttgaagtggtggcctaactacggctacactagaagaacagtatttggtatctgcgctctgctgaagccagttaccttcggaaaaagagttggtagctcttgatccggcaaacaaaccaccgctggtagcggtggtttttttgtttgcaagcagcagattacgcgcagaaaaaaaggatctcaagaagatcctttgatcttttctacggggtctgacgctcagtggaacgaaaactcacgttaagggattttggtcatgagattatcaaaaaggatcttcacctagatccttttaaattaaaaatgaagttttaaatcaatctaaagtatatatgagtaaacttggtctgacagttaccaatgcttaatcagtgaggcacctatctcagcgatctgtctatttcgttcatccatagttgcctgactccccgtcgtgtagataactacgatacgggagggcttaccatctggccccagtgctgcaatgataccgcgagaaccacgctcaccggctccagatttatcagcaataaaccagccagccggaagggccgagcgcagaagtggtcctgcaactttatccgcctccatccagtctattaattgttgccgggaagctagagtaagtagttcgccagttaatagtttgcgcaacgttgttgccattgctacaggcatcgtggtgtcacgctcgtcgtttggtatggcttcattcagctccggttcccaacgatcaaggcgagttacatgatcccccatgttgtgcaaaaaagcggttagctccttcggtcctccgatcgttgtcagaagtaagttggccgcagtgttatcactcatggttatggcagcactgcataattctcttactgtcatgccatccgtaagatgcttttctgtgactggtgagtactcaaccaagtcattctgagaatagtgtatgcggcgaccgagttgctcttgcccggcgtcaatacgggataataccgcgccacatagcagaactttaaaagtgctcatcattggaaaacgttcttcggggcgaaaactctcaaggatcttaccgctgttgagatccagttcgatgtaacccactcgtgcacccaactgatcttcagcatcttttactttcaccagcgtttctgggtgagcaaaaacaggaaggcaaaatgccgcaaaaaagggaataagggcgacacggaaatgttgaatactcatactcttcctttttcaatattattgaagcatttatcagggttattgtctcatgagcggatacatatttgaatgtatttagaaaaataaacaaataggggttccgcgcacatttccccgaaaagtgccac

SEQ ID NO: 87 - DNA, 2762 bp, Artificial Sequence
  HLA-C-sg-sp-4 vector V2.B.3
ctaaattgtaagcgttaatattttgttaaaattcgcgttaaatttttgttaaatcagctcattttttaaccaataggccgaaatcggcaaaatcccttataaatcaaaagaatagaccgagatagggttgagtggccgctacagggcgctcccattcgccattcaggctgcgcaactgttgggaagggcgtttcggtgcgggcctcttcgctattacgccagctggcgaaagggggatgtgctgcaaggcgattaagttgggtaacgccagggttttcccagtcacgacgttgtaaaacgacggccagtgagcgcgacgtaatacgactcactatagggcgaattggcggaaggccgtcaaggccgcatggatccaaggtcgggcaggaagagggcctatttcccatgattccttcatatttgcatatacgatacaaggctgttagagagataattagaattaatttgactgtaaacacaaagatattagtacaaaatacgtgacgtagaaagtaataatttcttgggtagtttgcagttttaaaattatgttttaaaatggactatcatatgcttaccgtaacttgaaagtatttcgatttcttggctttatatatcttgtggaaaggacgaaacaccggggccggagtattgggaccgtttaagagctatgctggaaacagcatagcaagtttaaataaggctagtccgttatcaacttgaaaaagtggcaccgagtcggtgctttttttcagacatccatagatctagctcgagttttttttctagactgggcctcatgggccttccgctcactgcccgctttccagtcgggaaacctgtcgtgccagctgcattaacatggtcatagctgtttccttgcgtattgggcgctctccgcttcctcgctcactgactcgctgcgctcggtcgttcgggtaaagcctggggtgcctaatgagcaaaaggccagcaaaaggccaggaaccgtaaaaaggccgcgttgctggcgtttttccataggctccgcccccctgacgagcatcacaaaaatcgacgctcaagtcagaggtggcgaaacccgacaggactataaagataccaggcgtttccccctggaagctccctcgtgcgctctcctgttccgaccctgccgcttaccggatacctgtccgcctttctcccttcgggaagcgtggcgctttctcatagctcacgctgtaggtatctcagttcggtgtaggtcgttcgctccaagctgggctgtgtgcacgaaccccccgttcagcccgaccgctgcgccttatccggtaactatcgtcttgagtccaacccggtaagacacgacttatcgccactggcagcagccactggtaacaggattagcagagcgaggtatgtaggcggtgctacagagttcttgaagtggtggcctaactacggctacactagaagaacagtatttggtatctgcgctctgctgaagccagttaccttcggaaaaagagttggtagctcttgatccggcaaacaaaccaccgctggtagcggtggtttttttgtttgcaagcagcagattacgcgcagaaaaaaaggatctcaagaagatcctttgatcttttctacggggtctgacgctcagtggaacgaaaactcacgttaagggattttggtcatgagattatcaaaaaggatcttcacctagatccttttaaattaaaaatgaagttttaaatcaatctaaagtatatatgagtaaacttggtctgacagttaccaatgcttaatcagtgaggcacctatctcagcgatctgtctatttcgttcatccatagttgcctgactccccgtcgtgtagataactacgatacgggagggcttaccatctggccccagtgctgcaatgataccgcgagaaccacgctcaccggctccagatttatcagcaataaaccagccagccggaagggccgagcgcagaagtggtcctgcaactttatccgcctccatccagtctattaattgttgccgggaagctagagtaagtagttcgccagttaatagtttgcgcaacgttgttgccattgctacaggcatcgtggtgtcacgctcgtcgtttggtatggcttcattcagctccggttcccaacgatcaaggcgagttacatgatcccccatgttgtgcaaaaaagcggttagctccttcggtcctccgatcgttgtcagaagtaagttggccgcagtgttatcactcatggttatggcagcactgcataattctcttactgtcatgccatccgtaagatgcttttctgtgactggtgagtactcaaccaagtcattctgagaatagtgtatgcggcgaccgagttgctcttgcccggcgtcaatacgggataataccgcgccacatagcagaactttaaaagtgctcatcattggaaaacgttcttcggggcgaaaactctcaaggatcttaccgctgttgagatccagttcgatgtaacccactcgtgcacccaactgatcttcagcatcttttactttcaccagcgtttctgggtgagcaaaaacaggaaggcaaaatgccgcaaaaaagggaataagggcgacacggaaatgttgaatactcatactcttcctttttcaatattattgaagcatttatcagggttattgtctcatgagcggatacatatttgaatgtatttagaaaaataaacaaataggggttccgcgcacatttccccgaaaagtgccac

SEQ ID NO: 88 - DNA, 2762 bp, Artificial Sequence
  HLA-A-ex2-3_sg-sp-opti_1 vector V2.I.10
ctaaattgtaagcgttaatattttgttaaaattcgcgttaaatttttgttaaatcagctcattttttaaccaataggccgaaatcggcaaaatcccttataaatcaaaagaatagaccgagatagggttgagtggccgctacagggcgctcccattcgccattcaggctgcgcaactgttgggaagggcgtttcggtgcgggcctcttcgctattacgccagctggcgaaagggggatgtgctgcaaggcgattaagttgggtaacgccagggttttcccagtcacgacgttgtaaaacgacggccagtgagcgcgacgtaatacgactcactatagggcgaattggcggaaggccgtcaaggccgcatggatccaaggtcgggcaggaagagggcctatttcccatgattccttcatatttgcatatacgatacaaggctgttagagagataattagaattaatttgactgtaaacacaaagatattagtacaaaatacgtgacgtagaaagtaataatttcttgggtagtttgcagttttaaaattatgttttaaaatggactatcatatgcttaccgtaacttgaaagtatttcgatttcttggctttatatatcttgtggaaaggacgaaacaccgtccccaggctctcactgaagtttaagagctatgctggaaacagcatagcaagtttaaataaggctagtccgttatcaacttgaaaaagtggcaccgagtcggtgctttttttcagacatccatagatctagctcgagttttttttctagactgggcctcatgggccttccgctcactgcccgctttccagtcgggaaacctgtcgtgccagctgcattaacatggtcatagctgtttccttgcgtattgggcgctctccgcttcctcgctcactgactcgctgcgctcggtcgttcgggtaaagcctggggtgcctaatgagcaaaaggccagcaaaaggccaggaaccgtaaaaaggccgcgttgctggcgtttttccataggctccgcccccctgacgagcatcacaaaaatcgacgctcaagtcagaggtggcgaaacccgacaggactataaagataccaggcgtttccccctggaagctccctcgtgcgctctcctgttccgaccctgccgcttaccggatacctgtccgcctttctcccttcgggaagcgtggcgctttctcatagctcacgctgtaggtatctcagttcggtgtaggtcgttcgctccaagctgggctgtgtgcacgaaccccccgttcagcccgaccgctgcgccttatccggtaactatcgtcttgagtccaacccggtaagacacgacttatcgccactggcagcagccactggtaacaggattagcagagcgaggtatgtaggcggtgctacagagttcttgaagtggtggcctaactacggctacactagaagaacagtatttggtatctgcgctctgctgaagccagttaccttcggaaaaagagttggtagctcttgatccggcaaacaaaccaccgctggtagcggtggtttttttgtttgcaagcagcagattacgcgcagaaaaaaaggatctcaagaagatcctttgatcttttctacggggtctgacgctcagtggaacgaaaactcacgttaagggattttggtcatgagattatcaaaaaggatcttcacctagatccttttaaattaaaaatgaagttttaaatcaatctaaagtatatatgagtaaacttggtctgacagttaccaatgcttaatcagtgaggcacctatctcagcgatctgtctatttcgttcatccatagttgcctgactccccgtcgtgtagataactacgatacgggagggcttaccatctggccccagtgctgcaatgataccgcgagaaccacgctcaccggctccagatttatcagcaataaaccagccagccggaagggccgagcgcagaagtggtcctgcaactttatccgcctccatccagtctattaattgttgccgggaagctagagtaagtagttcgccagttaatagtttgcgcaacgttgttgccattgctacaggcatcgtggtgtcacgctcgtcgtttggtatggcttcattcagctccggttcccaacgatcaaggcgagttacatgatcccccatgttgtgcaaaaaagcggttagctccttcggtcctccgatcgttgtcagaagtaagttggccgcagtgttatcactcatggttatggcagcactgcataattctcttactgtcatgccatccgtaagatgcttttctgtgactggtgagtactcaaccaagtcattctgagaatagtgtatgcggcgaccgagttgctcttgcccggcgtcaatacgggataataccgcgccacatagcagaactttaaaagtgctcatcattggaaaacgttcttcggggcgaaaactctcaaggatcttaccgctgttgagatccagttcgatgtaacccactcgtgcacccaactgatcttcagcatcttttactttcaccagcgtttctgggtgagcaaaaacaggaaggcaaaatgccgcaaaaaagggaataagggcgacacggaaatgttgaatactcatactcttcctttttcaatattattgaagcatttatcagggttattgtctcatgagcggatacatatttgaatgtatttagaaaaataaacaaataggggttccgcgcacatttccccgaaaagtgccac

SEQ ID NO: 89 - DNA, 2763 bp, Artificial Sequence
  HLA-A-ex2-3_sg-sp-opti_2 vector V2.J.1
ctaaattgtaagcgttaatattttgttaaaattcgcgttaaatttttgttaaatcagctcattttttaaccaataggccgaaatcggcaaaatcccttataaatcaaaagaatagaccgagatagggttgagtggccgctacagggcgctcccattcgccattcaggctgcgcaactgttgggaagggcgtttcggtgcgggcctcttcgctattacgccagctggcgaaagggggatgtgctgcaaggcgattaagttgggtaacgccagggttttcccagtcacgacgttgtaaaacgacggccagtgagcgcgacgtaatacgactcactatagggcgaattggcggaaggccgtcaaggccgcatggatccaaggtcgggcaggaagagggcctatttcccatgattccttcatatttgcatatacgatacaaggctgttagagagataattagaattaatttgactgtaaacacaaagatattagtacaaaatacgtgacgtagaaagtaataatttcttgggtagtttgcagttttaaaattatgttttaaaatggactatcatatgcttaccgtaacttgaaagtatttcgatttcttggctttatatatcttgtggaaaggacgaaacaccgcaggctctcactgaacgggagtttaagagctatgctggaaacagcatagcaagtttaaataaggctagtccgttatcaacttgaaaaagtggcaccgagtcggtgctttttttcagacatccatagatctagctcgagttttttttctagactgggcctcatgggccttccgctcactgcccgctttccagtcgggaaacctgtcgtgccagctgcattaacatggtcatagctgtttccttgcgtattgggcgctctccgcttcctcgctcactgactcgctgcgctcggtcgttcgggtaaagcctggggtgcctaatgagcaaaaggccagcaaaaggccaggaaccgtaaaaaggccgcgttgctggcgtttttccataggctccgcccccctgacgagcatcacaaaaatcgacgctcaagtcagaggtggcgaaacccgacaggactataaagataccaggcgtttccccctggaagctccctcgtgcgctctcctgttccgaccctgccgcttaccggatacctgtccgcctttctcccttcgggaagcgtggcgctttctcatagctcacgctgtaggtatctcagttcggtgtaggtcgttcgctccaagctgggctgtgtgcacgaaccccccgttcagcccgaccgctgcgccttatccggtaactatcgtcttgagtccaacccggtaagacacgacttatcgccactggcagcagccactggtaacaggattagcagagcgaggtatgtaggcggtgctacagagttcttgaagtggtggcctaactacggctacactagaagaacagtatttggtatctgcgctctgctgaagccagttaccttcggaaaaagagttggtagctcttgatccggcaaacaaaccaccgctggtagcggtggtttttttgtttgcaagcagcagattacgcgcagaaaaaaaggatctcaagaagatcctttgatcttttctacggggtctgacgctcagtggaacgaaaactcacgttaagggattttggtcatgagattatcaaaaaggatcttcacctagatccttttaaattaaaaatgaagttttaaatcaatctaaagtatatatgagtaaacttggtctgacagttaccaatgcttaatcagtgaggcacctatctcagcgatctgtctatttcgttcatccatagttgcctgactccccgtcgtgtagataactacgatacgggagggcttaccatctggccccagtgctgcaatgataccgcgagaaccacgctcaccggctccagatttatcagcaataaaccagccagccggaagggccgagcgcagaagtggtcctgcaactttatccgcctccatccagtctattaattgttgccgggaagctagagtaagtagttcgccagttaatagtttgcgcaacgttgttgccattgctacaggcatcgtggtgtcacgctcgtcgtttggtatggcttcattcagctccggttcccaacgatcaaggcgagttacatgatcccccatgttgtgcaaaaaagcggttagctccttcggtcctccgatcgttgtcagaagtaagttggccgcagtgttatcactcatggttatggcagcactgcataattctcttactgtcatgccatccgtaagatgcttttctgtgactggtgagtactcaaccaagtcattctgagaatagtgtatgcggcgaccgagttgctcttgcccggcgtcaatacgggataataccgcgccacatagcagaactttaaaagtgctcatcattggaaaacgttcttcggggcgaaaactctcaaggatcttaccgctgttgagatccagttcgatgtaacccactcgtgcacccaactgatcttcagcatcttttactttcaccagcgtttctgggtgagcaaaaacaggaaggcaaaatgccgcaaaaaagggaataagggcgacacggaaatgttgaatactcatactcttcctttttcaatattattgaagcatttatcagggttattgtctcatgagcggatacatatttgaatgtatttagaaaaataaacaaataggggttccgcgcacatttccccgaaaagtgccac

SEQ ID NO: 90 - DNA, 2762 bp, Artificial Sequence
  AAVSI_sg-sp-opti_3 vector V2.J.6
ctaaattgtaagcgttaatattttgttaaaattcgcgttaaatttttgttaaatcagctcattttttaaccaataggccgaaatcggcaaaatcccttataaatcaaaagaatagaccgagatagggttgagtggccgctacagggcgctcccattcgccattcaggctgcgcaactgttgggaagggcgtttcggtgcgggcctcttcgctattacgccagctggcgaaagggggatgtgctgcaaggcgattaagttgggtaacgccagggttttcccagtcacgacgttgtaaaacgacggccagtgagcgcgacgtaatacgactcactatagggcgaattggcggaaggccgtcaaggccgcatggatccaaggtcgggcaggaagagggcctatttcccatgattccttcatatttgcatatacgatacaaggctgttagagagataattagaattaatttgactgtaaacacaaagatattagtacaaaatacgtgacgtagaaagtaataatttcttgggtagtttgcagttttaaaattatgttttaaaatggactatcatatgcttaccgtaacttgaaagtatttcgatttcttggctttatatatcttgtggaaaggacgaaacaccgtcaccaatcctgtccctaggtttaagagctatgctggaaacagcatagcaagtttaaataaggctagtccgttatcaacttgaaaaagtggcaccgagtcggtgctttttttcagacatccatagatctagctcgagttttttttctagactgggcctcatgggccttccgctcactgcccgctttccagtcgggaaacctgtcgtgccagctgcattaacatggtcatagctgtttccttgcgtattgggcgctctccgcttcctcgctcactgactcgctgcgctcggtcgttcgggtaaagcctggggtgcctaatgagcaaaaggccagcaaaaggccaggaaccgtaaaaaggccgcgttgctggcgtttttccataggctccgcccccctgacgagcatcacaaaaatcgacgctcaagtcagaggtggcgaaacccgacaggactataaagataccaggcgtttccccctggaagctccctcgtgcgctctcctgttccgaccctgccgcttaccggatacctgtccgcctttctcccttcgggaagcgtggcgctttctcatagctcacgctgtaggtatctcagttcggtgtaggtcgttcgctccaagctgggctgtgtgcacgaaccccccgttcagcccgaccgctgcgccttatccggtaactatcgtcttgagtccaacccggtaagacacgacttatcgccactggcagcagccactggtaacaggattagcagagcgaggtatgtaggcggtgctacagagttcttgaagtggtggcctaactacggctacactagaagaacagtatttggtatctgcgctctgctgaagccagttaccttcggaaaaagagttggtagctcttgatccggcaaacaaaccaccgctggtagcggtggtttttttgtttgcaagcagcagattacgcgcagaaaaaaaggatctcaagaagatcctttgatcttttctacggggtctgacgctcagtggaacgaaaactcacgttaagggattttggtcatgagattatcaaaaaggatcttcacctagatccttttaaattaaaaatgaagttttaaatcaatctaaagtatatatgagtaaacttggtctgacagttaccaatgcttaatcagtgaggcacctatctcagcgatctgtctatttcgttcatccatagttgcctgactccccgtcgtgtagataactacgatacgggagggcttaccatctggccccagtgctgcaatgataccgcgagaaccacgctcaccggctccagatttatcagcaataaaccagccagccggaagggccgagcgcagaagtggtcctgcaactttatccgcctccatccagtctattaattgttgccgggaagctagagtaagtagttcgccagttaatagtttgcgcaacgttgttgccattgctacaggcatcgtggtgtcacgctcgtcgtttggtatggcttcattcagctccggttcccaacgatcaaggcgagttacatgatcccccatgttgtgcaaaaaagcggttagctccttcggtcctccgatcgttgtcagaagtaagttggccgcagtgttatcactcatggttatggcagcactgcataattctcttactgtcatgccatccgtaagatgcttttctgtgactggtgagtactcaaccaagtcattctgagaatagtgtatgcggcgaccgagttgctcttgcccggcgtcaatacgggataataccgcgccacatagcagaactttaaaagtgctcatcattggaaaacgttcttcggggcgaaaactctcaaggatcttaccgctgttgagatccagttcgatgtaacccactcgtgcacccaactgatcttcagcatcttttactttcaccagcgtttctgggtgagcaaaaacaggaaggcaaaatgccgcaaaaaagggaataagggcgacacggaaatgttgaatactcatactcttcctttttcaatattattgaagcatttatcagggttattgtctcatgagcggatacatatttgaatgtatttagaaaaataaacaaataggggttccgcgcacatttccccgaaaagtgccac

SEQ ID NO: 91 - DNA, 19 bp, Artificial Sequence
  TRAC-GT-F1 ddPCR primer/probe
atgtgcaaacgccttcaac

SEQ ID NO: 92 - DNA, 20 bp, Artificial Sequence
  TRAC-GT-R1 ddPCR primer/probe 1.F.8
ttcggaacccaatcactgac

SEQ ID NO: 93 - DNA, 26 bp, Artificial Sequence
  TRAC-probe-FAM ddPCR primer/probe
tttctcgaccagcttgacatcacagg

SEQ ID NO: 94 - DNA, 21 bp, Artificial Sequence
  TRBC2-GT-F1 ddPCR primer/probe 1.F.9
gctgtcaagtccagttctacg

SEQ ID NO: 95 - DNA, 20 bp, Artificial Sequence
  TRBC2-GT-R1 ddPCR primer/probe 1.F.10
cttgctggtaagactcggag

SEQ ID NO: 96 - DNA, 23 bp, Artificial Sequence
  TRBC2-probe-FAM ddPCR primer/probe 1.G.2
caaacccgtcacccagatcgtca

SEQ ID NO: 97 - DNA, 23 bp, Artificial Sequence
  TRAC-TCRA-ex1-F1 ddPCR primer/probe 10.A.9
ctgatcctcttgtcccacagata

SEQ ID NO: 98 - DNA, 26 bp, Artificial Sequence
  TRAC-TCRA-ex1-F1 ddPCR primer/probe 10.A.10
gacttgtcactggatttagagtctct

SEQ ID NO: 99 - DNA, 22 bp, Artificial Sequence
  TRAC-probe(HEX) ddPCR primer/probe 10.B.6
atccagaaccctgaccctgccg

SEQ ID NO: 100 - DNA, 18 bp, Homo sapiens
  HCMVpp65_GT_F2ddPCR primer/probe 21.I.1
tcgacgcccaaaaagcac

SEQ ID NO: 101 - DNA, 17 bp, Homo sapiens
  HCMVpp28_GT_F1 ddPCR primer/probe 21.I.2
tgcctccttgccctttg

SEQ ID NO: 102 - DNA, 19 bp, Homo sapiens
  HCMVpp52_GT_F1 ddPCR primer/probe 21.I.3
cgtccctaacaccaagaag

SEQ ID NO: 103 - DNA, 19 bp, Homo sapiens
  Myc-Tag_GT_R1 ddPCR primer/probe 20.H.10
aaggtcctcctcagagatg

SEQ ID NO: 104 - DNA, 27 bp, Homo sapiens
  Linker-Myc_Probe_Fam ddPCR primer/probe 20.H.9
cttttgttctccagatccagatccacc